European Patent Application EP 4 437 839 A1, published October 2, 2024. Title: COMPOSITIONS AND METHODS COMPRISING PLANTS WITH REDUCED RAFFINOSE FAMILY OLIGOSACCHARIDES AND/OR HIGH PROTEIN CONTENT. Applicant: Benson Hill, Inc. Application US. The sequence listing filed with the application follows.

SEQUENCE LISTING (52 sequences)

SEQ ID NO: 1 - DNA, 1745 bp, Pisum sativum
  source 1..1745: mol_type = genomic DNA
ttttttcaatttgcagataatttgaattgaagttatccaacattttccaaaaactttatattagagttgttgttacaatcctttatcaaaaagcatttgttatatattacaattacaaaagaagaaactaaatgaaaaaaataccataaataaaagcacaacaatatatacctgaaaatacaagccaagatacagacccatatgtacaaaaaccaaagatcaaattccccaaattagaacaaaacacacaaaactagaaatctatggaataactagaaatctatattccatttgactattagcaccgaccgcaaagtctggttgcacctcctcattcttattccaaaaaacagctcagttaagctgccgaaggtgctgtgacatatcgaacacgaccaacctccgacaacgcctgtacaaacggctcttcaacatcattcctttgtgtctcacaatttccactcaaattcttcttgtagtcaagtgaagaatcactgtatatatccaaccatttctgcaccaacatctttatatcctccctctgcatattctcttcttttccagtatacctccaaggctttgaaccctaaacaaaaaaacaacaaaccaatttaacagtgttcagttaataattgcgcagacatatacagtattcagttagtagtttcccagagacatatacttacggctgcacaatagtgaacaaccttgactttcctaagctcaacattctcaggatgacgccacaacatagcaagaacaagattataaaccaaaggaattggcctataaatatccttaaaatacatgttcaagaaatcttgttctgcaaacggagtaggagcagtaacttgacaagttttcaaaagatcatcataagtctcaacacttggctcaaacagaaacatgccagcattgaagtaaagggaaggaggttcacccatttctttcggccattgcaccttctccggacactgctgacagtacccgatcttatactgtggtgtatgactccatgttttttcacagaaacaatccatcacagcgtagaaataaccgtctggtagatcaaaaagatgatctatgttttcatatacctgaatgtctccatccaaatatatcatcttgctgtattccacaaactgcaacataagtattaaattataattcaattaattaatcaataataactttttttctctagaactaaaaaaaatgacacgtgtgtaataatagtgatgacgtggcagaataatagtatgtggaagtgtaagtgtacctcccatattcggagtttggagtaattgatgacgtaataagccatagcaaactgagtttgattttccggtgggtaaaccggttgaatctcacggacgatacatccttgagattccaacatctcacggtgctcctccggtacgtctggaagcacggcaacaaccagcgggtacgccgtttttacttttcgtaaaccttttgccaaacctattacgcctttcacgtagtcgccgttgccggcgagaaacgttacgtatgcacgtttcagtttcgtgaaaccggtaactggtttcgtagaggtctgaacgatctccggtgccatttttttgagtgctgaaaattgaaaactgtttagtttagagagtttggaaaactgtttattttagagaggatggttaatagtttgttcgatgattgtgagttgaatggtggaggtaaaggtggtatatataataaaaagggaggtg

SEQ ID NO: 2 - DNA, 1219 bp, Pisum sativum
  source 1..1219: mol_type = genomic DNA
atggctcctgatattgtaactgctgcaaccaccgtcaccgactctcaaactaagactgcaaaacgtgcttttgtcacgtttcttgccggaaacggcgactatgtgaaaggtgttgttggtttagcaaaaggtctccgtaaggtgaaaaccatgtaccctcttgtggttgcagtgttgcctgatgttccggtggaacaccggaatattctcatctcacaaggttgcattgttagagagatcgaacctgtttacccacctgagaacgaaactcagtttgctatggcttattatgttatcaactactccaaacttcgtatttgggctgtaagtatatataaactctgatgaattattatactgtgtaatcatattctaattacaaatttcaattttacagtttgaggaatatgagaagatgatttaccttgacggtgatatacaagttttcgaaaacattgaccatttatttgacttgccaaataactatttctatgctgtcatggattgtttttgtgaggccacatggggtcactccaagcaatatgaaatcggatactgtcaacaatgtcccgacaaggttgaatggcctagtagtgttggtcccaaaccacctctttacttcaatgctggcatgtttgtttatgaacctaatatggatacttatcatgatcttcttcaaaaacttcaagtgaataaaccaacttcctttgctgaacaggtaatattaatgtttaattagttactaaaaattgtgacttaattggattatgaagtgtgcttaataactttttattcatgttttgcaggattttttgaatatgtatttcaatgacaagtataagccaattcctaatgtttataatcttgtgctggctatgttgtggcgtcatcctgagaatgttgagcttgaaaaagttaaagttgttcattattgtgcagctgtaagttttcaatatttaacgattacaacttctataattacaacttaaaatttaattttcttaaattgggttaatttcagggttctaagccttggaggtacactggtgtggaggagaatatgcagagagaagatataaagatgctggtgaagaagtggtgggaggtgtatgaagatgaaagtttggattacaaggaagcgattaatacgaatcgcttaacatcagcaattttggaagctggtggtttcaactttgtccgcgcgccaaacgctgcttaa

SEQ ID NO: 3 - DNA, 3651 bp, Pisum sativum
  source 1..3651: mol_type = genomic DNA
atttttcaaatcataaatcaagaggctattcaaacattttttatatagttaaccctataaatatgtagggtctcttttctcaggctacacattttcaaccatagccaagttaaccatcaaattaagctcgtctctgactacgtcatctacctatagaaacattcctaccggttacttaaagctactaagctatctgagtctcatcaatcaccatggcaccaccaagcataaccaaaactgcaacccagcaagacgtaataagcaccgtcgatattggtaactcacccttgttgtccatatccttggaccaatcacgtaacttccttgtaaatggccatcctttcctcacccaagtcccacctaacataacaacaacaacaacatccaccccttccccttttctcgacttcaaatccaacaaagataccattgccaacaacaacaacaccttgcaacaacaaggttgtttcgttgggttcaacaccacggaagccaaaagccaccacgtggttccactcggcaaactaaaaggaatcaaattcacgagcatattccggttcaaagtttggtggacaactcactgggtcggaacaaacggacacgaactacaacacgaaacacaaatcttaatcctcgacaaaaacatctccctcggacgaccctacgttctcctcctcccaatcctcgaaaactccttccgaacctcactccaacccggcctcaacgattacgtcgacatgtccgtcgagagcggttcaacacatgtcaccgggtcaaccttcaaagcctgtctttacctccatctcagcaacgacccataccgtttagtgaaagaagcagtgaaagtaatccaaaccaagttagggacattcaagactctagaagaaaaaacaccacctagtatcatcgagaaattcggttggtgcacgtgggatgcgttttatttgaaggttcatccaaaaggtgtatgggaaggtgtgaaagctctcacagacggtggttgtcctccgggtttcgtcataatcgacgacggttggcaatccatttctcatgatgatgatgatcctgttacagagcgagatggaatgaaccgaacctcagctggggaacaaatgccatgcaggcttataaaatatgaagagaattataaatttagagaatacgaaaatggtgataatggagggaagaaaggtttggttggttttgtgagggatttgaaggaagagtttaggagtgttgagagtgtttatgtctggcatgcgctttgtgggtattggggtggggttagacctaaagtgtgtggaatgccggaagctaaggttgttgttccgaagctgtctccgggggtgaagatgacgatggaggatttagcggtggataagattgttgagaatggtgtggggctagtgcctccaaatttggcgcaggagatgtttgatgggattcactctcatttggagtcggcgggaattgacggtgttaaagttgacgttatccatgtaagtcttataaaattctactcctataatttatgtcggtgcacgtatgatttatgtcggtgtgtcatgatatgagttgcatgagaattacaaatgagcacgtacgttttgttgttgttgctgtggtcctaaattatgattttactcggtggtgaaaaggtttactacactttgcaatttttgtgtgaaaaatattctgactcgattattgtaatttagctacatttgttttgttctagtttgcaataatagttttacacgacaaggcaactatgaatacgtagcggtggttcatttcatttaaatttgtctactggtttgtgacatcatcacgatggacgtgaagtctcaaaacagtgtacacctacatacatgacagctatggtttaaattgtaactgcagggtttatatttgaaaatcacttgtctcgggtagaaatggatgtcgtcttgtacaacaaacaatagcatgatttttacagaaaaataaataaattagataagtttaagtaatgcttatgaatatgtattaaattgtttttataaatctctcaaatattacatcaaatgtttatattaattaaaaaattcaaataacgaaacaagtgtgatatctaatgtttaaatgatttcaaaatttaacacaatatttggtttatttccattttgtagttgcttgagttactatcagaggaatatggtggacgagttgagctagcaaaagcttattacaaagcactaacctcatcagtgaacaaacatttcaaaggcaatggtgtaattgcaagcatggagcattgcaatgacttctttctcctcggcacggaagccatatccctcggccgcgtcggagatgatttttggtgctgtgacccctctggtgatccaaatggtacatattggctccaaggttgtcacatggtacattgtgcctacaacagtttatggatgggaaatttcattcatccagattgggacatgtttcagtccactcatccttgtgccgaatttcacgccgcctcaagagccatctctggtggaccagtttacgttagtgattgcgttggtaatcacaatttcaagttgctcaaatcttttgttttgcccgacggttctatcttgcgttgtcaacattacgcactccctacacgagactgcttatttgaagaccctttgcataatggcaaaacaatgctcaaaatttggaatctcaacaaagtaagtttcatcttatcaaattttgtacatgacaagcgcgttatatgcatgtgtctgtttgcacgctagtattatatatgatattgatttttttagtagttaatttagaatgattttacagtatgctggtgttttgggtctattcaactgccaaggtggtgggtggtgtcctgagacacggcgaaacaagagcgcttctgaattttcacacgcggtgacatgttatgcaagtcctgaagatattgaatggtgcaatggaaaaaccccaatggacatcaaaggtgtggatgttttcgctgtgtattttttcaaggagaagaaactgagtctcatgaagtgttccgatagattggaagtttcgctcgagccatttagttttgagctaatgacagtgtctccgctgaaagtgttttcgaaaaggttgatacagtttgctccgattgggttagtgaacatgctgaactccggcggtgccgttcagtctctggagtttgatgatagtgcaagcttggtcaagattggggtgagaggttgtggggagttgagtgtttttgcgtctgagaaaccagtttgctgtaaaattgacggggttagtgtggaatttgattatgaggacaaaatggtgagagttcaaattctgtggcctggttcttcaacattgtctttggtcgagtttttattttgatccctcatgagaataacttgggatcctatatatgtgactgttttaaagtactttgtataagtgtgatgtgtatatattttcacttttaaatgtgtgtttgttttaataggattatgcagttaggtggttaattagttatttgtttttgaagtaactaagttacttgtgttgtaagccacacttatagaaattgatggggttagtgtggaatttgattccttgcaatggatgtgaattaaaattttgcac

SEQ ID NO: 4 - DNA, 1398 bp, Pisum sativum
  source 1..1398: mol_type = genomic DNA
atgtctcctccaaatccaaccttaaactcaaacaaaaacaacatcaccacaaccaaacaccttaattcttgttccaattcacccttcaccttcacgttatccgagtcaactctaaaagtcaacaatcacatcatcctctctgatgtccccaaaaacatcaccaccacaactacttccaccaccaccaccaccaccaacggttgcttcctcggcttcaaagccaccgattcgaaaagccgccatgtggcacccattggaaaactcaaaaacataaacttcacaagcatattccggttcaaagtatggtggtccactctttggaccggttcaaacggcaaagacatcgaaaccgaaactcaatttctcatgctccaaaactcggatccaaatccaggttcggatccaaacacgggtcggccctatgttttatttctccccataatagaaggtccatttcgcgcttctctgcaatccgatgaaaacgacaacgttttagtctgcgtcgagagtggttcaacttcaataacaaaatctcaatacgacactgtcgtttaccttcatgcaggtaacgatccatttaagctagtaaaagaagccatgaaaactgtgaggggccacttaggaactttcaagcttctagaagaaaaaactgtaccgggcatagtagagaaatttggatggtgtacatgggatgcattttatcttaaggtacaccctcaaggaatttgggaaggtgttaaaaatttaactaatggtggttgtccgcctggctttgttttaatcgacgatggttggcaatctatagcccacgatgatgatccgattaatactaacgatgggatcaatcgaacggacgcaggtgaacagatgccatgtaggttaattaaattcgaagagaattataaatttaaggattataagaatggattagggttaggtggatttgttaaggaattaaaaaaagattttgagagtgttgagtatgtgtatgtatggcatgctttgtgtggttattggggtgggataagacctggtgttgagggtttacctgaagctactgtggagaaacctaagttgaccgttggattagaaactactatggaagatttggctgtggataagattgttaataatggtgtagggttagttcctcctcatttggttgagcaaatgtatgaaggtcttcattctcttttggaagattctggaattgatggggtcaaagttgacgtcatccatgtaagtatttttatttttattttaacaactttttctttctttatactctttacggttctagtttttttagtttaataacgaaattaatttctttatcttaaattccagtcatttttatcctcttgtcacatatttgtactaaaaatagatgatttgtga

SEQ ID NO: 5 - DNA, 1005 bp, synthetic construct
  source 1..1005: mol_type = other DNA
atggcaccggagatcgttcagacctctacgaaaccagttaccggtttcacgaaactgaaacgtgcatacgtaacgtttctcgccggcaacggcgactacgtgaaaggcgtaataggtttggcaaaaggtttacgaaaagtaaaaacggcgtacccgctggttgttgccgtgcttccagacgtaccggaggagcaccgtgagatgttggaatctcaaggatgtatcgtccgtgagattcaaccggtttacccaccggaaaatcaaactcagtttgctatggcttattacgtcatcaattactccaaactccgaatatgggagtttgtggaatacagcaagatgatatatttggatggagacattcaggtatatgaaaacatagatcatctttttgatctaccagacggttatttctacgctgtgatggattgtttctgtgaaaaaacatggagtcatacaccacagtataagatcgggtactgtcagcagtgtccggagaaggtgcaatggccgaaagaaatgggtgaacctccttccctttacttcaatgctggcatgtttctgtttgagccaagtgttgagacttatgatgatcttttgaaaacttgtcaagttactgctcctactccgtttgcagaacaagatttcttgaacatgtattttaaggatatttataggccaattcctttggtttataatcttgttcttgctatgttgtggcgtcatcctgagaatgttgagcttaggaaagtcaaggttgttcactattgtgcagccggttcaaagccttggaggtatactggaaaagaagagaatatgcagagggaggatataaagatgttggtgcagaaatggttggatatatacagtgattcttcacttgactacaagaagaatttgagtggaaattgtgagacacaaaggaatgatgttgaagagccgtttgtacaggcgttgtcggaggttggtcgtgttcgatatgtcacagcaccttcggcagcttaa

SEQ ID NO: 6 - DNA, 978 bp, synthetic construct
  source 1..978: mol_type = other DNA
atggctcctgatattgtaactgctgcaaccaccgtcaccgactctcaaactaagactgcaaaacgtgcttttgtcacgtttcttgccggaaacggcgactatgtgaaaggtgttgttggtttagcaaaaggtctccgtaaggtgaaaaccatgtaccctcttgtggttgcagtgttgcctgatgttccggtggaacaccggaatattctcatctcacaaggttgcattgttagagagatcgaacctgtttacccacctgagaacgaaactcagtttgctatggcttattatgttatcaactactccaaacttcgtatttgggcttttgaggaatatgagaagatgatttaccttgacggtgatatacaagttttcgaaaacattgaccatttatttgacttgccaaataactatttctatgctgtcatggattgtttttgtgaggccacatggggtcactccaagcaatatgaaatcggatactgtcaacaatgtcccgacaaggttgaatggcctagtagtgttggtcccaaaccacctctttacttcaatgctggcatgtttgtttatgaacctaatatggatacttatcatgatcttcttcaaaaacttcaagtgaataaaccaacttcctttgctgaacaggattttttgaatatgtatttcaatgacaagtataagccaattcctaatgtttataatcttgtgctggctatgttgtggcgtcatcctgagaatgttgagcttgaaaaagttaaagttgttcattattgtgcagctggttctaagccttggaggtacactggtgtggaggagaatatgcagagagaagatataaagatgctggtgaagaagtggtgggaggtgtatgaagatgaaagtttggattacaaggaagcgattaatacgaatcgcttaacatcagcaattttggaagctggtggtttcaactttgtccgcgcgccaaacgctgcttaa

SEQ ID NO: 7 - DNA, 2397 bp, synthetic construct
  source 1..2397: mol_type = other DNA
atggcaccaccaagcataaccaaaactgcaacccagcaagacgtaataagcaccgtcgatattggtaactcacccttgttgtccatatccttggaccaatcacgtaacttccttgtaaatggccatcctttcctcacccaagtcccacctaacataacaacaacaacaacatccaccccttccccttttctcgacttcaaatccaacaaagataccattgccaacaacaacaacaccttgcaacaacaaggttgtttcgttgggttcaacaccacggaagccaaaagccaccacgtggttccactcggcaaactaaaaggaatcaaattcacgagcatattccggttcaaagtttggtggacaactcactgggtcggaacaaacggacacgaactacaacacgaaacacaaatcttaatcctcgacaaaaacatctccctcggacgaccctacgttctcctcctcccaatcctcgaaaactccttccgaacctcactccaacccggcctcaacgattacgtcgacatgtccgtcgagagcggttcaacacatgtcaccgggtcaaccttcaaagcctgtctttacctccatctcagcaacgacccataccgtttagtgaaagaagcagtgaaagtaatccaaaccaagttagggacattcaagactctagaagaaaaaacaccacctagtatcatcgagaaattcggttggtgcacgtgggatgcgttttatttgaaggttcatccaaaaggtgtatgggaaggtgtgaaagctctcacagacggtggttgtcctccgggtttcgtcataatcgacgacggttggcaatccatttctcatgatgatgatgatcctgttacagagcgagatggaatgaaccgaacctcagctggggaacaaatgccatgcaggcttataaaatatgaagagaattataaatttagagaatacgaaaatggtgataatggagggaagaaaggtttggttggttttgtgagggatttgaaggaagagtttaggagtgttgagagtgtttatgtctggcatgcgctttgtgggtattggggtggggttagacctaaagtgtgtggaatgccggaagctaaggttgttgttccgaagctgtctccgggggtgaagatgacgatggaggatttagcggtggataagattgttgagaatggtgtggggctagtgcctccaaatttggcgcaggagatgtttgatgggattcactctcatttggagtcggcgggaattgacggtgttaaagttgacgttatccatttgcttgagttactatcagaggaatatggtggacgagttgagctagcaaaagcttattacaaagcactaacctcatcagtgaacaaacatttcaaaggcaatggtgtaattgcaagcatggagcattgcaatgacttctttctcctcggcacggaagccatatccctcggccgcgtcggagatgatttttggtgctgtgacccctctggtgatccaaatggtacatattggctccaaggttgtcacatggtacattgtgcctacaacagtttatggatgggaaatttcattcatccagattgggacatgtttcagtccactcatccttgtgccgaatttcacgccgcctcaagagccatctctggtggaccagtttacgttagtgattgcgttggtaatcacaatttcaagttgctcaaatcttttgttttgcccgacggttctatcttgcgttgtcaacattacgcactccctacacgagactgcttatttgaagaccctttgcataatggcaaaacaatgctcaaaatttggaatctcaacaaatatgctggtgttttgggtctattcaactgccaaggtggtgggtggtgtcctgagacacggcgaaacaagagcgcttctgaattttcacacgcggtgacatgttatgcaagtcctgaagatattgaatggtgcaatggaaaaaccccaatggacatcaaaggtgtggatgttttcgctgtgtattttttcaaggagaagaaactgagtctcatgaagtgttccgatagattggaagtttcgctcgagccatttagttttgagctaatgacagtgtctccgctgaaagtgttttcgaaaaggttgatacagtttgctccgattgggttagtgaacatgctgaactccggcggtgccgttcagtctctggagtttgatgatagtgcaagcttggtcaagattggggtgagaggttgtggggagttgagtgtttttgcgtctgagaaaccagtttgctgtaaaattgacggggttagtgtggaatttgattatgaggacaaaatggtgagagttcaaattctgtggcctggttcttcaacattgtctttggtcgagtttttattttga

SEQ ID NO: 8 - DNA, 1290 bp, synthetic construct
  source 1..1290: mol_type = other DNA
atgtctcctccaaatccaaccttaaactcaaacaaaaacaacatcaccacaaccaaacaccttaattcttgttccaattcacccttcaccttcacgttatccgagtcaactctaaaagtcaacaatcacatcatcctctctgatgtccccaaaaacatcaccaccacaactacttccaccaccaccaccaccaccaacggttgcttcctcggcttcaaagccaccgattcgaaaagccgccatgtggcacccattggaaaactcaaaaacataaacttcacaagcatattccggttcaaagtatggtggtccactctttggaccggttcaaacggcaaagacatcgaaaccgaaactcaatttctcatgctccaaaactcggatccaaatccaggttcggatccaaacacgggtcggccctatgttttatttctccccataatagaaggtccatttcgcgcttctctgcaatccgatgaaaacgacaacgttttagtctgcgtcgagagtggttcaacttcaataacaaaatctcaatacgacactgtcgtttaccttcatgcaggtaacgatccatttaagctagtaaaagaagccatgaaaactgtgaggggccacttaggaactttcaagcttctagaagaaaaaactgtaccgggcatagtagagaaatttggatggtgtacatgggatgcattttatcttaaggtacaccctcaaggaatttgggaaggtgttaaaaatttaactaatggtggttgtccgcctggctttgttttaatcgacgatggttggcaatctatagcccacgatgatgatccgattaatactaacgatgggatcaatcgaacggacgcaggtgaacagatgccatgtaggttaattaaattcgaagagaattataaatttaaggattataagaatggattagggttaggtggatttgttaaggaattaaaaaaagattttgagagtgttgagtatgtgtatgtatggcatgctttgtgtggttattggggtgggataagacctggtgttgagggtttacctgaagctactgtggagaaacctaagttgaccgttggattagaaactactatggaagatttggctgtggataagattgttaataatggtgtagggttagttcctcctcatttggttgagcaaatgtatgaaggtcttcattctcttttggaagattctggaattgatggggtcaaagttgacgtcatccattcatttttatcctcttgtcacatatttgtactaaaaatagatgatttgtga

SEQ ID NO: 9 - protein, 334 aa, Pisum sativum
MAPEIVQTSTKPVTGFTKLKRAYVTFLAGNGDYVKGVIGLAKGLRKVKTAYPLVVAVLPDVPEEHREMLESQGCIVREIQPVYPPENQTQFAMAYYVINYSKLRIWEFVEYSKMIYLDGDIQVYENIDHLFDLPDGYFYAVMDCFCEKTWSHTPQYKIGYCQQCPEKVQWPKEMGEPPSLYFNAGMFLFEPSVETYDDLLKTCQVTAPTPFAEQDFLNMYFKDIYRPIPLVYNLVLAMLWRHPENVELRKVKVVHYCAAGSKPWRYTGKEENMQREDIKMLVQKWLDIYSDSSLDYKKNLSGNCETQRNDVEEPFVQALSEVGRVRYVTAPSAA

SEQ ID NO: 10 - protein, 325 aa, Pisum sativum
MAPDIVTAATTVTDSQTKTAKRAFVTFLAGNGDYVKGVVGLAKGLRKVKTMYPLVVAVLPDVPVEHRNILISQGCIVREIEPVYPPENETQFAMAYYVINYSKLRIWAFEEYEKMIYLDGDIQVFENIDHLFDLPNNYFYAVMDCFCEATWGHSKQYEIGYCQQCPDKVEWPSSVGPKPPLYFNAGMFVYEPNMDTYHDLLQKLQVNKPTSFAEQDFLNMYFNDKYKPIPNVYNLVLAMLWRHPENVELEKVKVVHYCAAGSKPWRYTGVEENMQREDIKMLVKKWWEVYEDESLDYKEAINTNRLTSAILEAGGFNFVRAPNAA

SEQ ID NO: 11 - protein, 798 aa, Pisum sativum
MAPPSITKTATQQDVISTVDIGNSPLLSISLDQSRNFLVNGHPFLTQVPPNITTTTTSTPSPFLDFKSNKDTIANNNNTLQQQGCFVGFNTTEAKSHHVVPLGKLKGIKFTSIFRFKVWWTTHWVGTNGHELQHETQILILDKNISLGRPYVLLLPILENSFRTSLQPGLNDYVDMSVESGSTHVTGSTFKACLYLHLSNDPYRLVKEAVKVIQTKLGTFKTLEEKTPPSIIEKFGWCTWDAFYLKVHPKGVWEGVKALTDGGCPPGFVIIDDGWQSISHDDDDPVTERDGMNRTSAGEQMPCRLIKYEENYKFREYENGDNGGKKGLVGFVRDLKEEFRSVESVYVWHALCGYWGGVRPKVCGMPEAKVVVPKLSPGVKMTMEDLAVDKIVENGVGLVPPNLAQEMFDGIHSHLESAGIDGVKVDVIHLLELLSEEYGGRVELAKAYYKALTSSVNKHFKGNGVIASMEHCNDFFLLGTEAISLGRVGDDFWCCDPSGDPNGTYWLQGCHMVHCAYNSLWMGNFIHPDWDMFQSTHPCAEFHAASRAISGGPVYVSDCVGNHNFKLLKSFVLPDGSILRCQHYALPTRDCLFEDPLHNGKTMLKIWNLNKYAGVLGLFNCQGGGWCPETRRNKSASEFSHAVTCYASPEDIEWCNGKTPMDIKGVDVFAVYFFKEKKLSLMKCSDRLEVSLEPFSFELMTVSPLKVFSKRLIQFAPIGLVNMLNSGGAVQSLEFDDSASLVKIGVRGCGELSVFASEKPVCCKIDGVSVEFDYEDKMVRVQILWPGSSTLSLVEFLF

SEQ ID NO: 12 - protein, 429 aa, Pisum sativum
MSPPNPTLNSNKNNITTTKHLNSCSNSPFTFTLSESTLKVNNHIILSDVPKNITTTTTSTTTTTTNGCFLGFKATDSKSRHVAPIGKLKNINFTSIFRFKVWWSTLWTGSNGKDIETETQFLMLQNSDPNPGSDPNTGRPYVLFLPIIEGPFRASLQSDENDNVLVCVESGSTSITKSQYDTVVYLHAGNDPFKLVKEAMKTVRGHLGTFKLLEEKTVPGIVEKFGWCTWDAFYLKVHPQGIWEGVKNLTNGGCPPGFVLIDDGWQSIAHDDDPINTNDGINRTDAGEQMPCRLIKFEENYKFKDYKNGLGLGGFVKELKKDFESVEYVYVWHALCGYWGGIRPGVEGLPEATVEKPKLTVGLETTMEDLAVDKIVNNGVGLVPPHLVEQMYEGLHSLLEDSGIDGVKVDVIHSFLSSCHIFVLKIDDL

SEQ ID NO: 13 - DNA, 28 bp, synthetic construct
  source 1..28: mol_type = other DNA
taataggtttggcaaaaggtttacgaaa

SEQ ID NO: 14 - DNA, 28 bp, synthetic construct
  source 1..28: mol_type = other DNA
ggagtcggcgggaattgacggtgttaaa

SEQ ID NO: 15 - DNA, 1005 bp, synthetic construct
  source 1..1005: mol_type = other DNA
atggcaccggagatcgttcagacctctacgaaaccagttaccggtttcacgaaactgaaacgtgcatacgtaacgtttctcgccggcaacggcgactacgtgaaaggcgtaataggtttggcaaaagatttacgaaaagtaaaaacggcgtacccgctggttgttgccgtgcttccagacgtaccggaggagcaccgtgagatgttggaatctcaaggatgtatcgtccgtgagattcaaccggtttacccaccggaaaatcaaactcagtttgctatggcttattacgtcatcaattactccaaactccgaatatgggagtttgtggaatacagcaagatgatatatttggatggagacattcaggtatatgaaaacatagatcatctttttgatctaccagacggttatttctacgctgtgatggattgtttctgtgaaaaaacatggagtcatacaccacagtataagatcgggtactgtcagcagtgtccggagaaggtgcaatggccgaaagaaatgggtgaacctccttccctttacttcaatgctggcatgtttctgtttgagccaagtgttgagacttatgatgatcttttgaaaacttgtcaagttactgctcctactccgtttgcagaacaagatttcttgaacatgtattttaaggatatttataggccaattcctttggtttataatcttgttcttgctatgttgtggcgtcatcctgagaatgttgagcttaggaaagtcaaggttgttcactattgtgcagccggttcaaagccttggaggtatactggaaaagaagagaatatgcagagggaggatataaagatgttggtgcagaaatggttggatatatacagtgattcttcacttgactacaagaagaatttgagtggaaattgtgagacacaaaggaatgatgttgaagagccgtttgtacaggcgttgtcggaggttggtcgtgttcgatatgtcacagcaccttcggcagcttaa

SEQ ID NO: 16 - DNA, 2397 bp, synthetic construct
  source 1..2397: mol_type = other DNA
atggcaccaccaagcataaccaaaactgcaacccagcaagacgtaataagcaccgtcgatattggtaactcacccttgttgtccatatccttggaccaatcacgtaacttccttgtaaatggccatcctttcctcacccaagtcccacctaacataacaacaacaacaacatccaccccttccccttttctcgacttcaaatccaacaaagataccattgccaacaacaacaacaccttgcaacaacaaggttgtttcgttgggttcaacaccacggaagccaaaagccaccacgtggttccactcggcaaactaaaaggaatcaaattcacgagcatattccggttcaaagtttggtggacaactcactgggtcggaacaaacggacacgaactacaacacgaaacacaaatcttaatcctcgacaaaaacatctccctcggacgaccctacgttctcctcctcccaatcctcgaaaactccttccgaacctcactccaacccggcctcaacgattacgtcgacatgtccgtcgagagcggttcaacacatgtcaccgggtcaaccttcaaagcctgtctttacctccatctcagcaacgacccataccgtttagtgaaagaagcagtgaaagtaatccaaaccaagttagggacattcaagactctagaagaaaaaacaccacctagtatcatcgagaaattcggttggtgcacgtgggatgcgttttatttgaaggttcatccaaaaggtgtatgggaaggtgtgaaagctctcacagacggtggttgtcctccgggtttcgtcataatcgacgacggttggcaatccatttctcatgatgatgatgatcctgttacagagcgagatggaatgaaccgaacctcagctggggaacaaatgccatgcaggcttataaaatatgaagagaattataaatttagagaatacgaaaatggtgataatggagggaagaaaggtttggttggttttgtgagggatttgaaggaagagtttaggagtgttgagagtgtttatgtctgacatgcgctttgtgggtattggggtggggttagacctaaagtgtgtggaatgccggaagctaaggttgttgttccgaagctgtctccgggggtgaagatgacgatggaggatttagcggtggataagattgttgagaatggtgtggggctagtgcctccaaatttggcgcaggagatgtttgatgggattcactctcatttggagtcggcgggaattgacggtgttaaagttgacgttatccatttgcttgagttactatcagaggaatatggtggacgagttgagctagcaaaagcttattacaaagcactaacctcatcagtgaacaaacatttcaaaggcaatggtgtaattgcaagcatggagcattgcaatgacttctttctcctcggcacggaagccatatccctcggccgcgtcggagatgatttttggtgctgtgacccctctggtgatccaaatggtacatattggctccaaggttgtcacatggtacattgtgcctacaacagtttatggatgggaaatttcattcatccagattgggacatgtttcagtccactcatccttgtgccgaatttcacgccgcctcaagagccatctctggtggaccagtttacgttagtgattgcgttggtaatcacaatttcaagttgctcaaatcttttgttttgcccgacggttctatcttgcgttgtcaacattacgcactccctacacgagactgcttatttgaagaccctttgcataatggcaaaacaatgctcaaaatttggaatctcaacaaatatgctggtgttttgggtctattcaactgccaaggtggtgggtggtgtcctgagacacggcgaaacaagagcgcttctgaattttcacacgcggtgacatgttatgcaagtcctgaagatattgaatggtgcaatggaaaaaccccaatggacatcaaaggtgtggatgttttcgctgtgtattttttcaaggagaagaaactgagtctcatgaagtgttccgatagattggaagtttcgctcgagccatttagttttgagctaatgacagtgtctccgctgaaagtgttttcgaaaaggttgatacagtttgctccgattgggttagtgaacatgctgaactccggcggtgccgttcagtctctggagtttgatgatagtgcaagcttggtcaagattggggtgagaggttgtggggagttgagtgtttttgcgtctgagaaaccagtttgctgtaaaattgacggggttagtgtggaatttgattatgaggacaaaatggtgagagttcaaattctgtggcctggttcttcaacattgtctttggtcgagtttttattttga

SEQ ID NO: 17 - protein, 334 aa, synthetic construct
MAPEIVQTSTKPVTGFTKLKRAYVTFLAGNGDYVKGVIGLAKDLRKVKTAYPLVVAVLPDVPEEHREMLESQGCIVREIQPVYPPENQTQFAMAYYVINYSKLRIWEFVEYSKMIYLDGDIQVYENIDHLFDLPDGYFYAVMDCFCEKTWSHTPQYKIGYCQQCPEKVQWPKEMGEPPSLYFNAGMFLFEPSVETYDDLLKTCQVTAPTPFAEQDFLNMYFKDIYRPIPLVYNLVLAMLWRHPENVELRKVKVVHYCAAGSKPWRYTGKEENMQREDIKMLVQKWLDIYSDSSLDYKKNLSGNCETQRNDVEEPFVQALSEVGRVRYVTAPSAA

SEQ ID NO: 18 - protein, 347 aa, synthetic construct
MAPPSITKTATQQDVISTVDIGNSPLLSISLDQSRNFLVNGHPFLTQVPPNITTTTTSTPSPFLDFKSNKDTIANNNNTLQQQGCFVGFNTTEAKSHHVVPLGKLKGIKFTSIFRFKVWWTTHWVGTNGHELQHETQILILDKNISLGRPYVLLLPILENSFRTSLQPGLNDYVDMSVESGSTHVTGSTFKACLYLHLSNDPYRLVKEAVKVIQTKLGTFKTLEEKTPPSIIEKFGWCTWDAFYLKVHPKGVWEGVKALTDGGCPPGFVIIDDGWQSISHDDDDPVTERDGMNRTSAGEQMPCRLIKYEENYKFREYENGDNGGKKGLVGFVRDLKEEFRSVESVYV

SEQ ID NO: 19 - DNA, 15 bp, synthetic construct
  source 1..15: mol_type = other DNA
ggagatcgttcagac

SEQ ID NO: 20 - DNA, 16 bp, synthetic construct
  source 1..16: mol_type = other DNA
taagtgtacctcccat

SEQ ID NO: 21 - DNA, 16 bp, synthetic construct
  source 1..16: mol_type = other DNA
tggttggttttgtgag

SEQ ID NO: 22 - DNA, 16 bp, synthetic construct
  source 1..16: mol_type = other DNA
cgctaaatcctccatc

SEQ ID NO: 23 - DNA, 21 bp, synthetic construct
  source 1..21: mol_type = other DNA
gatgacgatggaggatttagc

SEQ ID NO: 24 - DNA, 21 bp, synthetic construct
  source 1..21: mol_type = other DNA
gcaccgacataaattatagga

SEQ ID NO: 25 - DNA, 1242 bp, Pisum sativum
  source 1..1242: mol_type = genomic DNA
atggcaccggagatcgttcagacctctacgaaaccagttaccggtttcacgaaactgaaacgtgcatacgtaacgtttctcgccggcaacggcgactacgtgaaaggcgtaataggtttggcaaaaggtttacgaaaagtaaaaacggcgtacccgctggttgttgccgtgcttccagacgtaccggaggagcaccgtgagatgttggaatctcaaggatgtatcgtccgtgagattcaaccggtttacccaccggaaaatcaaactcagtttgctatggcttattacgtcatcaattactccaaactccgaatatgggaggtacacttacacttccacatactattattctgccacgtcatcactattattacacacgtgtcattttttttagttctagagaaaaaaagttattattgattaattaattgaattataatttaatacttatgttgcagtttgtggaatacagcaagatgatatatttggatggagacattcaggtatatgaaaacatagatcatctttttgatctaccagacggttatttctacgctgtgatggattgtttctgtgaaaaaacatggagtcatacaccacagtataagatcgggtactgtcagcagtgtccggagaaggtgcaatggccgaaagaaatgggtgaacctccttccctttacttcaatgctggcatgtttctgtttgagccaagtgttgagacttatgatgatcttttgaaaacttgtcaagttactgctcctactccgtttgcagaacaagatttcttgaacatgtattttaaggatatttataggccaattcctttggtttataatcttgttcttgctatgttgtggcgtcatcctgagaatgttgagcttaggaaagtcaaggttgttcactattgtgcagccgtaagtatatgtctctgggaaactactaactgaatactgtatatgtctgcgcaattattaactgaacactgttaaattggtttgttgtttttttgtttagggttcaaagccttggaggtatactggaaaagaagagaatatgcagagggaggatataaagatgttggtgcagaaatggttggatatatacagtgattcttcacttgactacaagaagaatttgagtggaaattgtgagacacaaaggaatgatgttgaagagccgtttgtacaggcgttgtcggaggttggtcgtgttcgatatgtcacagcaccttcggcagcttaa

SEQ ID NO: 26 - DNA, 1242 bp, synthetic construct
  source 1..1242: mol_type = other DNA
atggcaccggagatcgttcagacctctacgaaaccagttaccggtttcacgaaactgaaacgtgcatacgtaacgtttctcgccggcaacggcgactacgtgaaaggcgtaataggtttggcaaaagatttacgaaaagtaaaaacggcgtacccgctggttgttgccgtgcttccagacgtaccggaggagcaccgtgagatgttggaatctcaaggatgtatcgtccgtgagattcaaccggtttacccaccggaaaatcaaactcagtttgctatggcttattacgtcatcaattactccaaactccgaatatgggaggtacacttacacttccacatactattattctgccacgtcatcactattattacacacgtgtcattttttttagttctagagaaaaaaagttattattgattaattaattgaattataatttaatacttatgttgcagtttgtggaatacagcaagatgatatatttggatggagacattcaggtatatgaaaacatagatcatctttttgatctaccagacggttatttctacgctgtgatggattgtttctgtgaaaaaacatggagtcatacaccacagtataagatcgggtactgtcagcagtgtccggagaaggtgcaatggccgaaagaaatgggtgaacctccttccctttacttcaatgctggcatgtttctgtttgagccaagtgttgagacttatgatgatcttttgaaaacttgtcaagttactgctcctactccgtttgcagaacaagatttcttgaacatgtattttaaggatatttataggccaattcctttggtttataatcttgttcttgctatgttgtggcgtcatcctgagaatgttgagcttaggaaagtcaaggttgttcactattgtgcagccgtaagtatatgtctctgggaaactactaactgaatactgtatatgtctgcgcaattattaactgaacactgttaaattggtttgttgtttttttgtttagggttcaaagccttggaggtatactggaaaagaagagaatatgcagagggaggatataaagatgttggtgcagaaatggttggatatatacagtgattcttcacttgactacaagaagaatttgagtggaaattgtgagacacaaaggaatgatgttgaagagccgtttgtacaggcgttgtcggaggttggtcgtgttcgatatgtcacagcaccttcggcagcttaa

SEQ ID NO: 27 - DNA, 1237 bp, synthetic construct
  source 1..1237: mol_type = other DNA
atggcaccggagatcgttcagacctctacgaaaccagttaccggtttcacgaaactgaaacgtgcatacgtaacgtttctcgccggcaacggcgactacgtgaaaggcgtaataggcaaaaggtttacgaaaagtaaaaacggcgtacccgctggttgttgccgtgcttccagacgtaccggaggagcaccgtgagatgttggaatctcaaggatgtatcgtccgtgagattcaaccggtttacccaccggaaaatcaaactcagtttgctatggcttattacgtcatcaattactccaaactccgaatatgggaggtacacttacacttccacatactattattctgccacgtcatcactattattacacacgtgtcattttttttagttctagagaaaaaaagttattattgattaattaattgaattataatttaatacttatgttgcagtttgtggaatacagcaagatgatatatttggatggagacattcaggtatatgaaaacatagatcatctttttgatctaccagacggttatttctacgctgtgatggattgtttctgtgaaaaaacatggagtcatacaccacagtataagatcgggtactgtcagcagtgtccggagaaggtgcaatggccgaaagaaatgggtgaacctccttccctttacttcaatgctggcatgtttctgtttgagccaagtgttgagacttatgatgatcttttgaaaacttgtcaagttactgctcctactccgtttgcagaacaagatttcttgaacatgtattttaaggatatttataggccaattcctttggtttataatcttgttcttgctatgttgtggcgtcatcctgagaatgttgagcttaggaaagtcaaggttgttcactattgtgcagccgtaagtatatgtctctgggaaactactaactgaatactgtatatgtctgcgcaattattaactgaacactgttaaattggtttgttgtttttttgtttagggttcaaagccttggaggtatactggaaaagaagagaatatgcagagggaggatataaagatgttggtgcagaaatggttggatatatacagtgattcttcacttgactacaagaagaatttgagtggaaattgtgagacacaaaggaatgatgttgaagagccgtttgtacaggcgttgtcggaggttggtcgtgttcgatatgtcacagcaccttcggcagcttaa

SEQ ID NO: 28 - DNA, 1235 bp, synthetic construct
  source 1..1235: mol_type = other DNA
atggcaccggagatcgttcagacctctacgaaaccagttaccggtttcacgaaactgaaacgtgcatacgtaacgtttctcgccggcaacggcgactacgtgaaaggcgtttggcaaaaggtttacgaaaagtaaaaacggcgtacccgctggttgttgccgtgcttccagacgtaccggaggagcaccgtgagatgttggaatctcaaggatgtatcgtccgtgagattcaaccggtttacccaccggaaaatcaaactcagtttgctatggcttattacgtcatcaattactccaaactccgaatatgggaggtacacttacacttccacatactattattctgccacgtcatcactattattacacacgtgtcattttttttagttctagagaaaaaaagttattattgattaattaattgaattataatttaatacttatgttgcagtttgtggaatacagcaagatgatatatttggatggagacattcaggtatatgaaaacatagatcatctttttgatctaccagacggttatttctacgctgtgatggattgtttctgtgaaaaaacatggagtcatacaccacagtataagatcgggtactgtcagcagtgtccggagaaggtgcaatggccgaaagaaatgggtgaacctccttccctttacttcaatgctggcatgtttctgtttgagccaagtgttgagacttatgatgatcttttgaaaacttgtcaagttactgctcctactccgtttgcagaacaagatttcttgaacatgtattttaaggatatttataggccaattcctttggtttataatcttgttcttgctatgttgtggcgtcatcctgagaatgttgagcttaggaaagtcaaggttgttcactattgtgcagccgtaagtatatgtctctgggaaactactaactgaatactgtatatgtctgcgcaattattaactgaacactgttaaattggtttgttgtttttttgtttagggttcaaagccttggaggtatactggaaaagaagagaatatgcagagggaggatataaagatgttggtgcagaaatggttggatatatacagtgattcttcacttgactacaagaagaatttgagtggaaattgtgagacacaaaggaatgatgttgaagagccgtttgtacaggcgttgtcggaggttggtcgtgttcgatatgtcacagcaccttcggcagcttaa

SEQ ID NO: 29 - protein, 64 aa, synthetic construct
MAPEIVQTSTKPVTGFTKLKRAYVTFLAGNGDYVKGVIGKRFTKSKNGVPAGCCRASRRTGGAP

SEQ ID NO: 30 - protein, 44 aa, synthetic construct
MAPEIVQTSTKPVTGFTKLKRAYVTFLAGNGDYVKGVWQKVYEK

SEQ ID NO: 31 - DNA, 3190 bp, Pisum sativum
  source 1..3190: mol_type = genomic DNA
atggcaccaccaagcataaccaaaactgcaacccagcaagacgtaataagcaccgtcgatattggtaactcacccttgttgtccatatccttggaccaatcacgtaacttccttgtaaatggccatcctttcctcacccaagtcccacctaacataacaacaacaacaacatccaccccttccccttttctcgacttcaaatccaacaaagataccattgccaacaacaacaacaccttgcaacaacaaggttgtttcgttgggttcaacaccacggaagccaaaagccaccacgtggttccactcggcaaactaaaaggaatcaaattcacgagcatattccggttcaaagtttggtggacaactcactgggtcggaacaaacggacacgaactacaacacgaaacacaaatcttaatcctcgacaaaaacatctccctcggacgaccctacgttctcctcctcccaatcctcgaaaactccttccgaacctcactccaacccggcctcaacgattacgtcgacatgtccgtcgagagcggttcaacacatgtcaccgggtcaaccttcaaagcctgtctttacctccatctcagcaacgacccataccgtttagtgaaagaagcagtgaaagtaatccaaaccaagttagggacattcaagactctagaagaaaaaacaccacctagtatcatcgagaaattcggttggtgcacgtgggatgcgttttatttgaaggttcatccaaaaggtgtatgggaaggtgtgaaagctctcacagacggtggttgtcctccgggtttcgtcataatcgacgacggttggcaatccatttctcatgatgatgatgatcctgttacagagcgagatggaatgaaccgaacctcagctggggaacaaatgccatgcaggcttataaaatatgaagagaattataaatttagagaatacgaaaatggtgataatggagggaagaaaggtttggttggttttgtgagggatttgaaggaagagtttaggagtgttgagagtgtttatgtctggcatgcgctttgtgggtattggggtggggttagacctaaagtgtgtggaatgccggaagctaaggttgttgttccgaagctgtctccgggggtgaagatgacgatggaggatttagcggtggataagattgttgagaatggtgtggggctagtgcctccaaatttggcgcaggagatgtttgatgggattcactctcatttggagtcggcgggaattgacggtgttaaagttgacgttatccatgtaagtcttataaaattctactcctataatttatgtcggtgcacgtatgatttatgtcggtgtgtcatgatatgagttgcatgagaattacaaatgagcacgtacgttttgttgttgttgctgtggtcctaaattatgattttactcggtggtgaaaaggtttactacactttgcaatttttgtgtgaaaaatattctgactcgattattgtaatttagctacatttgttttgttctagtttgcaataatagttttacacgacaaggcaactatgaatacgtagcggtggttcatttcatttaaatttgtctactggtttgtgacatcatcacgatggacgtgaagtctcaaaacagtgtacacctacatacatgacagctatggtttaaattgtaactgcagggtttatatttgaaaatcacttgtctcgggtagaaatggatgtcgtcttgtacaacaaacaatagcatgatttttacagaaaaataaataaattagataagtttaagtaatgcttatgaatatgtattaaattgtttttataaatctctcaaatattacatcaaatgtttatattaattaaaaaattcaaataacgaaacaagtgtgatatctaatgtttaaatgatttcaaaatttaacacaatatttggtttatttccattttgtagttgcttgagttactatcagaggaatatggtggacgagttgagctagcaaaagcttattacaaagcactaacctcatcagtgaacaaacatttcaaaggcaatggtgtaattgcaagcatggagcattgcaatgacttctttctcctcggcacggaagccatatccctcggccgcgtcggagatgatttttggtgctgtgacccctctggtgatccaaatggtacatattggctccaaggttgtcacatggtacattgtgcctacaacagtttatggatgggaaatttcattcatccagattgggacatgtttcagtccactcatccttgtgccgaatttcacgccgcctcaagagccatctctggtggaccagtttacgttagtgattgcgttggtaatcacaatttcaagttgctcaaatcttttgttttgcccgacggttctatcttgcgttgtcaacattacgcactccctacacgagactgcttatttgaagaccctttgcataatggcaaaacaatgctcaaaatttggaatctcaacaaagtaagtttcatcttatcaaattttgtacatgacaagcgcgttatatgcatgtgtctgtttgcacgctagtattatatatgatattgatttttttagtagttaatttagaatgattttacagtatgctggtgttttgggtctattcaactgccaaggtggtgggtggtgtcctgagacacggcgaaacaagagcgcttctgaattttcacacgcggtgacatgttatgcaagtcctgaagatattgaatggtgcaatggaaaaaccccaatggacatcaaaggtgtggatgttttcgctgtgtattttttcaaggagaagaaactgagtctcatgaagtgttccgatagattggaagtttcgctcgagccatttagttttgagctaatgacagtgtctccgctgaaagtgttttcgaaaaggttgatacagtttgctccgattgggttagtgaacatgctgaactccggcggtgccgttcagtctctggagtttgatgatagtgcaagcttggtcaagattggggtgagaggttgtggggagttgagtgtttttgcgtctgagaaaccagtttgctgtaaaattgacggggttagtgtggaatttgattatgaggacaaaatggtgagagttcaaattctgtggcctggttcttcaacattgtctttggtcgagtttttattttga

SEQ ID NO: 32 - DNA, 3190 bp, synthetic construct
  source 1..3190: mol_type = other DNA
atggcaccaccaagcataaccaaaactgcaacccagcaagacgtaataagcaccgtcgatattggtaactcacccttgttgtccatatccttggaccaatcacgtaacttccttgtaaatggccatcctttcctcacccaagtcccacctaacataacaacaacaacaacatccaccccttccccttttctcgacttcaaatccaacaaagataccattgccaacaacaacaacaccttgcaacaacaaggttgtttcgttgggttcaacaccacggaagccaaaagccaccacgtggttccactcggcaaactaaaaggaatcaaattcacgagcatattccggttcaaagtttggtggacaactcactgggtcggaacaaacggacacgaactacaacacgaaacacaaatcttaatcctcgacaaaaacatctccctcggacgaccctacgttctcctcctcccaatcctcgaaaactccttccgaacctcactccaacccggcctcaacgattacgtcgacatgtccgtcgagagcggttcaacacatgtcaccgggtcaaccttcaaagcctgtctttacctccatctcagcaacgacccataccgtttagtgaaagaagcagtgaaagtaatccaaaccaagttagggacattcaagactctagaagaaaaaacaccacctagtatcatcgagaaattcggttggtgcacgtgggatgcgttttatttgaaggttcatccaaaaggtgtatgggaaggtgtgaaagctctcacagacggtggttgtcctccgggtttcgtcataatcgacgacggttggcaatccatttctcatgatgatgatgatcctgttacagagcgagatggaatgaaccgaacctcagctggggaacaaatgccatgcaggcttataaaatatgaagagaattataaatttagagaatacgaaaatggtgataatggagggaagaaaggtttggttggttttgtgagggatttgaaggaagagtttaggagtgttgagagtgtttatgtctgacatgcgctttgtgggtattggggtggggttagacctaaagtgtgtggaatgccggaagctaaggttgttgttccgaagctgtctccgggggtgaagatgacgatggaggatttagcggtggataagattgttgagaatggtgtggggctagtgcctccaaatttggcgcaggagatgtttgatgggattcactctcatttggagtcggcgggaattgacggtgttaaagttgacgttatccatgtaagtcttataaaattctactcctataatttatgtcggtgcacgtatgatttatgtcggtgtgtcatgatatgagttgcatgagaattacaaatgagcacgtacgttttgttgttgttgctgtggtcctaaattatgattttactcggtggtgaaaaggtttactacactttgcaatttttgtgtgaaaaatattctgactcgattattgtaatttagctacatttgttttgttctagtttgcaataatagttttacacgacaaggcaactatgaatacgtagcggtggttcatttcatttaaatttgtctactggtttgtgacatcatcacgatggacgtgaagtctcaaaacagtgtacacctacatacatgacagctatggtttaaattgtaactgcagggtttatatttgaaaatcacttgtctcgggtagaaatggatgtcgtcttgtacaacaaacaatagcatgatttttacagaaaaataaataaattagataagtttaagtaatgcttatgaatatgtattaaattgtttttataaatctctcaaatattacatcaaatgtttatattaattaaaaaattcaaataacgaaacaagtgtgatatctaatgtttaaatgatttcaaaatttaacacaatatttggtttatttccattttgtagttgcttgagttactatcagaggaatatggtggacgagttgagctagcaaaagcttattacaaagcactaacctcatcagtgaacaaacatttcaaaggcaatggtgtaattgcaagcatggagcattgcaatgacttctttctcctcggcacggaagccatatccctcggccgcgtcggagatgatttttggtgctgtgacccctctggtgatccaaatggtacatattggctccaaggttgtcacatggtacattgtgcctacaacagtttatggatgggaaatttcattcatccagattgggacatgtttcagtccactcatccttgtgccgaatttcacgccgcctcaagagccatctctggtggaccagtttacgttagtgattgcgttggtaatcacaatttcaagttgctcaaatcttttgttttgcccgacggttctatcttgcgttgtcaacattacgcactccctacacgagactgcttatttgaagaccctttgcataatggcaaaacaatgctcaaaatttggaatctcaacaaagtaagtttcatcttatcaaattttgtacatgacaagcgcgttatatgcatgtgtctgtttgcacgctagtattatatatgatattgatttttttagtagttaatttagaatgattttacagtatgctggtgttttgggtctattcaactgccaaggtggtgggtggtgtcctgagacacggcgaaacaagagcgcttctgaattttcacacgcggtgacatgttatgcaagtcctgaagatattgaatggtgcaatggaaaaaccccaatggacatcaaaggtgtggatgttttcgctgtgtattttttcaaggagaagaaactgagtctcatgaagtgttccgatagattggaagtttcgctcgagccatttagttttgagctaatgacagtgtctccgctgaaagtgttttcgaaaaggttgatacagtttgctccgattgggttagtgaacatgctgaactccggcggtgccgttcagtctctggagtttgatgatagtgcaagcttggtcaagattggggtgagaggttgtggggagttgagtgtttttgcgtctgagaaaccagtttgctgtaaaattgacggggttagtgtggaatttgattatgaggacaaaatggtgagagttcaaattctgtggcctggttcttcaacattgtctttggtcgagtttttattttga

SEQ ID NO: 33 - DNA, 3182 bp, synthetic construct
  source 1..3182: mol_type = other DNA
atggcaccaccaagcataaccaaaactgcaacccagcaagacgtaataagcaccgtcgatattggtaactcacccttgttgtccatatccttggaccaatcacgtaacttccttgtaaatggccatcctttcctcacccaagtcccacctaacataacaacaacaacaacatccaccccttccccttttctcgacttcaaatccaacaaagataccattgccaacaacaacaacaccttgcaacaacaaggttgtttcgttgggttcaacaccacggaagccaaaagccaccacgtggttccactcggcaaactaaaaggaatcaaattcacgagcatattccggttcaaagtttggtggacaactcactgggtcggaacaaacggacacgaactacaacacgaaacacaaatcttaatcctcgacaaaaacatctccctcggacgaccctacgttctcctcctcccaatcctcgaaaactccttccgaacctcactccaacccggcctcaacgattacgtcgacatgtccgtcgagagcggttcaacacatgtcaccgggtcaaccttcaaagcctgtctttacctccatctcagcaacgacccataccgtttagtgaaagaagcagtgaaagtaatccaaaccaagttagggacattcaagactctagaagaaaaaacaccacctagtatcatcgagaaattcggttggtgcacgtgggatgcgttttatttgaaggttcatccaaaaggtgtatgggaaggtgtgaaagctctcacagacggtggttgtcctccgggtttcgtcataatcgacgacggttggcaatccatttctcatgatgatgatgatcctgttacagagcgagatggaatgaaccgaacctcagctggggaacaaatgccatgcaggcttataaaatatgaagagaattataaatttagagaatacgaaaatggtgataatggagggaagaaaggtttggttggttttgtgagggatttgaaggaagagtttaggagtgttgagagtgtttatgtctggcatgcgctttgtgggtattggggtggggttagacctaaagtgtgtggaatgccggaagctaaggttgttgttccgaagctgtctccgggggtgaagatgacgatggaggatttagcggtggataagattgttgagaatggtgtggggctagtgcctccaaatttggcgcaggagatgtttgatgggattcactctcatttggggaattgacggtgttaaagttgacgttatccatgtaagtcttataaaattctactcctataatttatgtcggtgcacgtatgatttatgtcggtgtgtcatgatatgagttgcatgagaattacaaatgagcacgtacgttttgttgttgttgctgtggtcctaaattatgattttactcggtggtgaaaaggtttactacactttgcaatttttgtgtgaaaaatattctgactcgattattgtaatttagctacatttgttttgttctagtttgcaataatagttttacacgacaaggcaactatgaatacgtagcggtggttcatttcatttaaatttgtctactggtttgtgacatcatcacgatggacgtgaagtctcaaaacagtgtacacctacatacatgacagctatggtttaaattgtaactgcagggtttatatttgaaaatcacttgtctcgggtagaaatggatgtcgtcttgtacaacaaacaatagcatgatttttacagaaaaataaataaattagataagtttaagtaatgcttatgaatatgtattaaattgtttttataaatctctcaaatattacatcaaatgtttatattaattaaaaaattcaaataacgaaacaagtgtgatatctaatgtttaaatgatttcaaaatttaacacaatatttggtttatttccattttgtagttgcttgagttactatcagaggaatatggtggacgagttgagctagcaaaagcttattacaaagcactaacctcatcagtgaacaaacatttcaaaggcaatggtgtaattgcaagcatggagcattgcaatgacttctttctcctcggcacggaagccatatccctcggccgcgtcggagatgatttttggtgctgtgacccctctggtgatccaaatggtacatattggctccaaggttgtcacatggtacattgtgcctacaacagtttatggatgggaaatttcattcatccagattgggacatgtttcagtccactcatccttgtgccgaatttcacgccgcctcaagagccatctctggtggaccagtttacgttagtgattgcgttggtaatcacaatttcaagttgctcaaatcttttgttttgcccgacggttctatcttgcgttgtcaacattacgcactccctacacgagactgcttatttgaagaccctttgcataatggcaaaacaatgctcaaaatttggaatctcaacaaagtaagtttcatcttatcaaattttgtacatgacaagcgcgttatatgcatgtgtctgtttgcacgctagtattatatatgatattgatttttttagtagttaatttagaatgattttacagtatgctggtgttttgggtctattcaactgccaaggtggtgggtggtgtcctgagacacggcgaaacaagagcgcttctgaattttcacacgcggtgacatgttatgcaagtcctgaagatattgaatggtgcaatggaaaaaccccaatggacatcaaaggtgtggatgttttcgctgtgtattttttcaaggagaagaaactgagtctcatgaagtgttccgatagattggaagtttcgctcgagccatttagttttgagctaatgacagtgtctccgctgaaagtgttttcgaaaaggttgatacagtttgctccgattgggttagtgaacatgctgaactccggcggtgccgttcagtctctggagtttgatgatagtgcaagcttggtcaagattggggtgagaggttgtggggagttgagtgtttttgcgtctgagaaaccagtttgctgtaaaattgacggggttagtgtggaatttgattatgaggacaaaatggtgagagttcaaattctgtggcctggttcttcaacattgtctttggtcgagtttttattttga

SEQ ID NO: 34 - DNA, 3183 bp, synthetic construct
  source 1..3183: mol_type = other DNA
atggcaccaccaagcataaccaaaactgcaacccagcaagacgtaataagcaccgtcgatattggtaactcacccttgttgtccatatccttggaccaatcacgtaacttccttgtaaatggccatcctttcctcacccaagtcccacctaacataacaacaacaacaacatccaccccttccccttttctcgacttcaaatccaacaaagataccattgccaacaacaacaacaccttgcaacaacaaggttgtttcgttgggttcaacaccacggaagccaaaagccaccacgtggttccactcggcaaactaaaaggaatcaaattcacgagcatattccggttcaaagtttggtggacaactcactgggtcggaacaaacggacacgaactacaacacgaaacacaaatcttaatcctcgacaaaaacatctccctcggacgaccctacgttctcctcctcccaatcctcgaaaactccttccgaacctcactccaacccggcctcaacgattacgtcgacatgtccgtcgagagcggttcaacacatgtcaccgggtcaaccttcaaagcctgtctttacctccatctcagcaacgacccataccgtttagtgaaagaagcagtgaaagtaatccaaaccaagttagggacattcaagactctagaagaaaaaacaccacctagtatcatcgagaaattcggttggtgcacgtgggatgcgttttatttgaaggttcatccaaaaggtgtatgggaaggtgtgaaagctctcacagacggtggttgtcctccgggtttcgtcataatcgacgacggttggcaatccatttctcatgatgatgatgatcctgttacagagcgagatggaatgaaccgaacctcagctggggaacaaatgccatgcaggcttataaaatatgaagagaattataaatttagagaatacgaaaatggtgataatggagggaagaaaggtttggttggttttgtgagggatttgaaggaagagtttaggagtgttgagagtgtttatgtctggcatgcgctttgtgggtattggggtggggttagacctaaagtgtgtggaatgccggaagctaaggttgttgttccgaagctgtctccgggggtgaagatgacgatggaggatttagcggtggataagattgttgagaatggtgtggggctagtgcctccaaatttggcgcaggagatgtttgatgggattcactctcatttggaggaattgacggtgttaaagttgacgttatccatgtaagtcttataaaattctactcctataatttatgtcggtgcacgtatgatttatgtcggtgtgtcatgatatgagttgcatgagaattacaaatgagcacgtacgttttgttgttgttgctgtggtcctaaattatgattttactcggtggtgaaaaggtttactacactttgcaatttttgtgtgaaaaatattctgactcgattattgtaatttagctacatttgttttgttctagtttgcaataatagttttacacgacaaggcaactatgaatacgtagcggtggttcatttcatttaaatttgtctactggtttgtgacatcatcacgatggacgtgaagtctcaaaacagtgtacacctacatacatgacagctatggtttaaattgtaactgcagggtttatatttgaaaatcacttgtctcgggtagaaatggatgtcgtcttgtacaacaaacaatagcatgatttttacagaaaaataaataaattagataagtttaagtaatgcttatgaatatgtattaaattgtttttataaatctctcaaatattacatcaaatgtttatattaattaaaaaattcaaataacgaaacaagtgtgatatctaatgtttaaatgatttcaaaatttaacacaatatttggtttatttccattttgtagttgcttgagttactatcagaggaatatggtggacgagttgagctagcaaaagcttattacaaagcactaacctcatcagtgaacaaacatttcaaaggcaatggtgtaattgcaagcatggagcattgcaatgacttctttctcctcggcacggaagccatatccctcggccgcgtcggagatgatttttggtgctgtgacccctctggtgatccaaatggtacatattggctccaaggttgtcacatggtacattgtgcctacaacagtttatggatgggaaatttcattcatccagattgggacatgtttcagtccactcatccttgtgccgaatttcacgccgcctcaagagccatctctggtggaccagtttacgttagtgattgcgttggtaatcacaatttcaagttgctcaaatcttttgttttgcccgacggttctatcttgcgttgtcaacattacgcactccctacacgagactgcttatttgaagaccctttgcataatggcaaaacaatgctcaaaatttggaatctcaacaaagtaagtttcatcttatcaaattttgtacatgacaagcgcgttatatgcatgtgtctgtttgcacgctagtattatatatgatattgatttttttagtagttaatttagaatgattttacagtatgctggtgttttgggtctattcaactgccaaggtggtgggtggtgtcctgagacacggcgaaacaagagcgcttctgaattttcacacgcggtgacatgttatgcaagtcctgaagatattgaatggtgcaatggaaaaaccccaatggacatcaaaggtgtggatgttttcgctgtgtattttttcaaggagaagaaactgagtctcatgaagtgttccgatagattggaagtttcgctcgagccatttagttttgagctaatgacagtgtctccgctgaaagtgttttcgaaaaggttgatacagtttgctccgattgggttagtgaacatgctgaactccggcggtgccgttcagtctctggagtttgatgatagtgcaagcttggtcaagattggggtgagaggttgtggggagttgagtgtttttgcgtctgagaaaccagtttgctgtaaaattgacggggttagtgtggaatttgattatgaggacaaaatggtgagagttcaaattctgtggcctggttcttcaacattgtctttggtcgagtttttattttga

SEQ ID NO: 35 - protein, 417 aa, synthetic construct
MAPPSITKTATQQDVISTVDIGNSPLLSISLDQSRNFLVNGHPFLTQVPPNITTTTTSTPSPFLDFKSNKDTIANNNNTLQQQGCFVGFNTTEAKSHHVVPLGKLKGIKFTSIFRFKVWWTTHWVGTNGHELQHETQILILDKNISLGRPYVLLLPILENSFRTSLQPGLNDYVDMSVESGSTHVTGSTFKACLYLHLSNDPYRLVKEAVKVIQTKLGTFKTLEEKTPPSIIEKFGWCTWDAFYLKVHPKGVWEGVKALTDGGCPPGFVIIDDGWQSISHDDDDPVTERDGMNRTSAGEQMPCRLIKYEENYKFREYENGDNGGKKGLVGFVRDLKEEFRSVESVYVWHALCGYWGGVRPKVCGMPEAKVVVPKLSPGVKMTMEDLAVDKIVENGVGLVPPNLAQEMFDGIHSHLGN

SEQ ID NO: 36 - protein, 425 aa, synthetic construct
MAPPLNSTTSNLIKTESIFDLSERKFKVKGFPPPNITTTTTSTPSPFLDFKSNKDTIANNNNTLQQQGCFVGFNTTEAKSHHVVPLGKLKGIKFTSIFRFKVWWTTHWVGTNGHELQHETQILILDKNISLGRPYVLLLPILENSFRTSLQPGLNDYVDMSVESGSTHVTGSTFKACLYLHLSNDPYRLVKEAVKVIQTKLGTFKTLEEKTPPSIIEKFGWCTWDAFYLKVHPKGVWEGVKALTDGGCPPGFVIIDDGWQSISHDDDDPVTERDGMNRTSAGEQMPCRLIKYEENYKFREYENGDNGGKKGLVGFVRDLKEEFRSVESVYVWHALCGYWGGVRPKVCGMPEAKVVVPKLSPGVKMTMEDLAVDKIVENGVGLVPPNLAQEMFDGIHSHLEELTVLKLTLSICLSYYQRNMVDELS

SEQ ID NO: 37 - DNA, 1709 bp, Pisum sativum
  source 1..1709: mol_type = genomic DNA
cacctccctttttattatatatacctcctttacctccaccattcaactcacaatcatcaaacaaactattaaccatcctctctaaaataaacagttttccaaactctctaaactaaacagttttcaattttcagcactcaaaaaaatggcaccggagatcgttcagacctctacgaaaccagttaccggtttcacgaaactgaaacgtgcatacgtaacgtttctcgccggcaacggcgactacgtgaaaggcgtaataggtttggcaaaaggtttacgaaaagtaaaaacggcgtacccgctggttgttgccgtgcttccagacgtaccggaggagcaccgtgagatgttggaatctcagggatgtatcgtccgtgagattcaaccggtttacccaccggaaaatcaaactcagtttgctatggcttattacgtcatcaattactccaaactccgtatatgggaggtagacttacacttacacattctattattttgccacgtcattactacttattacacgtgtcatttttttagatctatagaaaaaaagttattattgattaattaattgaaacttatgttgcagtttgtggaatacagcaagatgatatatttggatggagacattcaggtatatgaaaacatagatcatctttttgatctaccagacggttatttctacgctgtgatggattgtttctgtgaaaaaacatggagtcatacaccacagtataagattgggtactgtcagcagtgtccggagaaggtgcaatggccgaaagaaatgggtgaacctccttcactttacttcaatgctggcatgtttctgtttgagccaagtgttgagacttatgatgatcttttgaaaacttgtcaagttactgctcctactccgtttgcagaacaagatttcttgaacatgtattttaaggatatttataggccaattcctttggtttataatcttgttcttgctatgttgtggcgtcatcctgagaatgttgagcttaggaaagtcaaggttgttcactattgtgcagctgtaagtatatgtctctgtgcaattgtatatgtctctgcgcaattattaactgaatattaactgaacacttttaaattggtttgttgtttttgtttagggttcaaagccttggaggtatactggaaaagaagagaatatgcagagggaggatataaagatgttggtgcagaaatggttggatatatacagtgattcttcacttgactacaagaagaatttgagtggaaattgtgagacacaaaggaatgatgttgaagagccgtttgtacaggcgttgtcggaggttggtcgtgttcgatatgtcacagcaccttcggcagcttaactgagctgtttttaggaataagaatgaggaggtgcaaccagactttgcggtcggtgctaatagtcaaatggaatatagatttctagttttgtgtgttttgttctaatttggggaatttgatctttggtttttgtacatatgggtctgtatcttggcttgtattttcaggtatatattgttgtgcttttatttatggtatttttttcatttagtttcttcttttgtaattgtaatatataacaaatgctttttgataaaggattgtaacaacaactctaatataaagtttttggaaaatgttggataacttcaattcaaattatctgcaaattgaaaaaa

SEQ ID NO: 38 - DNA, 1005 bp, synthetic construct
  source 1..1005: mol_type = other DNA
atggcaccggagatcgttcagacctctacgaaaccagttaccggtttcacgaaactgaaacgtgcatacgtaacgtttctcgccggcaacggcgactacgtgaaaggcgtaataggtttggcaaaaggtttacgaaaagtaaaaacggcgtacccgctggttgttgccgtgcttccagacgtaccggaggagcaccgtgagatgttggaatctcagggatgtatcgtccgtgagattcaaccggtttacccaccggaaaatcaaactcagtttgctatggcttattacgtcatcaattactccaaactccgtatatgggagtttgtggaatacagcaagatgatatatttggatggagacattcaggtatatgaaaacatagatcatctttttgatctaccagacggttatttctacgctgtgatggattgtttctgtgaaaaaacatggagtcatacaccacagtataagattgggtactgtcagcagtgtccggagaaggtgcaatggccgaaagaaatgggtgaacctccttcactttacttcaatgctggcatgtttctgtttgagccaagtgttgagacttatgatgatcttttgaaaacttgtcaagttactgctcctactccgtttgcagaacaagatttcttgaacatgtattttaaggatatttataggccaattcctttggtttataatcttgttcttgctatgttgtggcgtcatcctgagaatgttgagcttaggaaagtcaaggttgttcactattgtgcagctggttcaaagccttggaggtatactggaaaagaagagaatatgcagagggaggatataaagatgttggtgcagaaatggttggatatatacagtgattcttcacttgactacaagaagaatttgagtggaaattgtgagacacaaaggaatgatgttgaagagccgtttgtacaggcgttgtcggaggttggtcgtgttcgatatgtcacagcaccttcggcagcttaa

SEQ ID NO: 39 - DNA, 4645 bp, Pisum sativum
  source 1..4645: mol_type = genomic DNA
aaaaaaataatcatgtatttaagtttactataaatacagagttcgagatattaaattgacaacgatttaaataatattaaaataaaaaaaaagtattttagaatagaaaaaataaaaacaaaaagaagaaaaggaaagatagaaagacacgcacaccaactttaaaaacaccacaaaataaaaaggtgacactaatatcaaaaccaaccttcaccacaccttcggttgggtcccactcagtgcatcacaattcattttcttttcatctataaatacacttcaatttcttgcttattcaaaaccaagcacaaacaagttgttattcacttcatcactatacaccacactaacaccattcttccattttcaattaattacccaaacctcaaaaaaatgtctcctccaaatccaaccttaaactcaaacaaaaacaacatcaccacaaccaaacaccttaattcttgttccaattcacccttcaccttcacgttatccgagtcaactctaaaagtcaacaatcacatcatcctctctgatgtccccaaaaacatcaccaccacaactacttccaccaccaccaccaccaccaacggttgcttcctcggcttcaaagccaccgattcgaaaagccgccatgtggcacccattggaaaactcaaaaacataaacttcacaagcatattccggttcaaagtatggtggtccactctttggaccggttcaaacggcaaagacatcgaaaccgaaactcaatttctcatgctccaaaactcggatccaaatccaggttcggatccaaacacgggtcggccctatgttttatttctccccataatagaaggtccatttcgcgcttctctgcaatccgatgaaaacgacaacgttttagtctgcgtcgagagtggttcaacttcaataacaaaatctcaatacgacactgtcgtttaccttcatgcaggtaacgatccatttaagctagtaaaagaagccatgaaaactgtgaggggccacttaggaactttcaagcttctagaagaaaaaactgtaccgggcatagtagagaaatttggatggtgtacatgggatgcattttatcttaaggtacaccctcaaggaatttgggaaggtgttaaaaatttaactaatggtggttgtccgcctggctttgttttaatcgacgatggttggcaatctatagcccacgatgatgatccgattaatactaacgatgggatcaatcgaacggacgcaggtgaacagatgccatgtaggttaattaaattcgaagagaattataaatttaaggattataagaatggattagggttaggtggatttgttaaggaattaaaaaaagattttgagagtgttgagtatgtgtatgtatggcatgctttgtgtggttattggggtgggataagacctggtgttgagggtttacctgaagctactgtggagaaacctaagttgaccgttggattagaaactactatggaagatttggctgtggataagattgttaataatggtgtagggttagttcctcctcatttggttgagcaaatgtatgaaggtcttcattctcttttggaagattctggaattgatggggtcaaagttgacgtcatccatgtaagtatttttatttttattttaacaactttttctttctttatactctttacggttctagtttttttagtttaataacgaaattaatttctttatcttaaattccagtcatttttatcctcttgtcacatatttgtactaaaaatagatgatttgtgaaatttttaatgaggtgttccttgtcaaatgtgacacatcattatataaattcatgtggaatgtgacatgtcaaccatataactgagatgtaagaggatgaaaaagtaattaatattttcttaatatactttattaaaaataagtttgactaataattataattatatatgtattaaaatttatttatttatttattcatatcatattttatgtgatcatatatttattgtttagtatggttattattctcttaagaaatatatatatatatatatatatataatatttatatatatatatatatatatatatatatatatattatatataatatatatatatattattatataaatataatatatatatatatatatatatatatatatatatatataattattatatatatatatatatttgtttcatattttcatgagatattgatcttagagaattataaaaaaaattaaaataatatgtaactcttttttaattagtggataaaattataaattattaaaaaccactcaatattttaactgaatggaaataaggtgttaaatatatattttaaatcccttcttacattttatatatatatatatatatatatatatatatatatatatatatatatataatatatatatatataaaatatatatattatatatatatataaagttatttagtttatgtcggcatgtttcacaaattaaggcataaaataaggtcaaactgtagggccaatttcattatccataatgttttggtcggcacgttatctttgtatttttaaattaaattgaaatattcacttttagaatgtcaaggcaggacaagctttttctttattgactttactattattttacaatgtatttagatttttttaaggaaaaaaattatacatcgaccgaatataaattattttaatgacataatatattaataaatttttattgaatggttttgacattttcttttttggttgatatattttataatcagttgctagagatggtgtgtgagaaatatggtggaagagttgatttagcaaaagcatattacaaagctctcacaacttcagtgaagaaacatttcaatggtaatggtgtcattgctagcatggagcattgcaatgatttcatgttacttggaaccgaagccatatccctcggtcgtgtcggtatgtcacacaaaccaactttcttaccttaaccagtaatacacacatgcatctacacatgacacttatatattaactactaatacacaatgcatgtacacatgacacatatatgtatctgcacatgtatctccacgtgacactttcatttgtgttgtgtacgaaaaaaaaccttaattaaaaaaatttgatttacttttctaggtgatgatttttggtgcactgacccttctggtgatccaaatgggacatattggttacaaggatgtcacatggtgcattgtgcatataatagtttatggatgggaaatttcattcaaccagattgggatatgtttcaatctacacacccttgtgcaactttccatgcagcttctagagccatatctggtggacctatttacataagtgacactgttggaaatcacaattttgaacttcttaagaccttagctttgccagatggtactatccttagatgtgaatattatgccctaccaactaaggattgtctctttgctgaccctttacatgatggcaaaacaatgctcaaaatatggaacctcaataaggtgaaccttccctcctcactttcataacaatatattctaatttgaatttgaattcatctcaatttccggtcatatcattatcggcgtgtagaaactatgagtcctaatcttctacggtctatttgattttgcaatcagacgtagggtttaaggagttggagatccagagttcaatctgcgtttaatataatattaactattgctaatttgtgattaaaaaatattcatctttcacaatctgcgtttgataatgtttttttttttttgtaatagtacaccggagttcttggtgtgtttaactgtcaaggaggaggatggtttcgtgacataagatcaaacaaatgtgcatctgaattttctcatttggtttcaactaagatcaacatcaaagacattgaatgggaaagtgggaaaaatccaatttccattgaaagtgtacaactttttgctctatatttcagccaagccaaaaagctcaaactattctctccatctgacactgaagagatctccttagaaccattcaattttgagcttataactgtttctcctatcactttatttcctaaaaagtccttgaagtttgctcctattggtttggtgaatatgttaaacaatggaggggcaattcagtcatttgaatttgatgaggataaagatttgattaaagttggagttagaggaagtggtgaaatgagagtgtttgcatcagagaaaccaaagatttgtagaattgatggcaaagaagttggttttgaatatgaagatttcatggttgtgattcaagtaccatggcctagttcttccaaattttcttctgttcagtatatattttgagcattggattagattatggacactttcaaacttatgattttgttttggtttttacataggacaatgtttaagttaaggggctttttgtttatcccttatttggattttgttgtataacttgctttttagttctaccttactaccttactagtatgtgaagaaataagttagtgagggatttaactattgtatcatttagaaaagctattttattgctttacttaaaaaagaatattaattataaaatattttt

SEQ ID NO: 40 - DNA, 2349 bp, synthetic construct
  source 1..2349: mol_type = other DNA
atgtctcctccaaatccaaccttaaactcaaacaaaaacaacatcaccacaaccaaacaccttaattcttgttccaattcacccttcaccttcacgttatccgagtcaactctaaaagtcaacaatcacatcatcctctctgatgtccccaaaaacatcaccaccacaactacttccaccaccaccaccaccaccaacggttgcttcctcggcttcaaagccaccgattcgaaaagccgccatgtggcacccattggaaaactcaaaaacataaacttcacaagcatattccggttcaaagtatggtggtccactctttggaccggttcaaacggcaaagacatcgaaaccgaaactcaatttctcatgctccaaaactcggatccaaatccaggttcggatccaaacacgggtcggccctatgttttatttctccccataatagaaggtccatttcgcgcttctctgcaatccgatgaaaacgacaacgttttagtctgcgtcgagagtggttcaacttcaataacaaaatctcaatacgacactgtcgtttaccttcatgcaggtaacgatccatttaagctagtaaaagaagccatgaaaactgtgaggggccacttaggaactttcaagcttctagaagaaaaaactgtaccgggcatagtagagaaatttggatggtgtacatgggatgcattttatcttaaggtacaccctcaaggaatttgggaaggtgttaaaaatttaactaatggtggttgtccgcctggctttgttttaatcgacgatggttggcaatctatagcccacgatgatgatccgattaatactaacgatgggatcaatcgaacggacgcaggtgaacagatgccatgtaggttaattaaattcgaagagaattataaatttaaggattataagaatggattagggttaggtggatttgttaaggaattaaaaaaagattttgagagtgttgagtatgtgtatgtatggcatgctttgtgtggttattggggtgggataagacctggtgttgagggtttacctgaagctactgtggagaaacctaagttgaccgttggattagaaactactatggaagatttggctgtggataagattgttaataatggtgtagggttagttcctcctcatttggttgagcaaatgtatgaaggtcttcattctcttttggaagattctggaattgatggggtcaaagttgacgtcatccatttgctagagatggtgtgtgagaaatatggtggaagagttgatttagcaaaagcatattacaaagctctcacaacttcagtgaagaaacatttcaatggtaatggtgtcattgctagcatggagcattgcaatgatttcatgttacttggaaccgaagccatatccctcggtcgtgtcggtgatgatttttggtgcactgacccttctggtgatccaaatgggacatattggttacaaggatgtcacatggtgcattgtgcatataatagtttatggatgggaaatttcattcaaccagattgggatatgtttcaatctacacacccttgtgcaactttccatgcagcttctagagccatatctggtggacctatttacataagtgacactgttggaaatcacaattttgaacttcttaagaccttagctttgccagatggtactatccttagatgtgaatattatgccctaccaactaaggattgtctctttgctgaccctttacatgatggcaaaacaatgctcaaaatatggaacctcaataagtacaccggagttcttggtgtgtttaactgtcaaggaggaggatggtttcgtgacataagatcaaacaaatgtgcatctgaattttctcatttggtttcaactaagatcaacatcaaagacattgaatgggaaagtgggaaaaatccaatttccattgaaagtgtacaactttttgctctatatttcagccaagccaaaaagctcaaactattctctccatctgacactgaagagatctccttagaaccattcaattttgagcttataactgtttctcctatcactttatttcctaaaaagtccttgaagtttgctcctattggtttggtgaatatgttaaacaatggaggggcaattcagtcatttgaatttgatgaggataaagatttgattaaagttggagttagaggaagtggtgaaatgagagtgtttgcatcagagaaaccaaagatttgtagaattgatggcaaagaagttggttttgaatatgaagatttcatggttgtgattcaagtaccatggcctagttcttccaaattttcttctgttcagtatatattttga

SEQ ID NO: 41 - protein, 782 aa, Pisum sativum
MSPPNPTLNSNKNNITTTKHLNSCSNSPFTFTLSESTLKVNNHIILSDVPKNITTTTTSTTTTTTNGCFLGFKATDSKSRHVAPIGKLKNINFTSIFRFKVWWSTLWTGSNGKDIETETQFLMLQNSDPNPGSDPNTGRPYVLFLPIIEGPFRASLQSDENDNVLVCVESGSTSITKSQYDTVVYLHAGNDPFKLVKEAMKTVRGHLGTFKLLEEKTVPGIVEKFGWCTWDAFYLKVHPQGIWEGVKNLTNGGCPPGFVLIDDGWQSIAHDDDPINTNDGINRTDAGEQMPCRLIKFEENYKFKDYKNGLGLGGFVKELKKDFESVEYVYVWHALCGYWGGIRPGVEGLPEATVEKPKLTVGLETTMEDLAVDKIVNNGVGLVPPHLVEQMYEGLHSLLEDSGIDGVKVDVIHLLEMVCEKYGGRVDLAKAYYKALTTSVKKHFNGNGVIASMEHCNDFMLLGTEAISLGRVGDDFWCTDPSGDPNGTYWLQGCHMVHCAYNSLWMGNFIQPDWDMFQSTHPCATFHAASRAISGGPIYISDTVGNHNFELLKTLALPDGTILRCEYYALPTKDCLFADPLHDGKTMLKIWNLNKYTGVLGVFNCQGGGWFRDIRSNKCASEFSHLVSTKINIKDIEWESGKNPISIESVQLFALYFSQAKKLKLFSPSDTEEISLEPFNFELITVSPITLFPKKSLKFAPIGLVNMLNNGGAIQSFEFDEDKDLIKVGVRGSGEMRVFASEKPKICRIDGKEVGFEYEDFMVVIQVPWPSSSKFSSVQYIF

SEQ ID NO: 42 - DNA, 2718 bp, Glycine max
  source 1..2718: mol_type = genomic DNA
atgccacctaacatcaccaccgttgttgccaatgtcaccaccgagcaattacccaaggctcgtggaggaagtgggcgtgccttcgtgacctttcttgctgggaacggtgattacgtaaagggtgtcgtgggtttggccaaaggactgagaaaggccaaaagcatgtaccctttggtggttgctgtgttaccagatgttcctgaagaacatcgtgagattctcaaatcccaaggttgcattgtcagggagattgaacctgtgtaccctcctgagaaccagacccagttcgccatggcctattatgtcatcaattactccaagctacgtatttgggaggtatacacatatcttaactcttttgttttttagtttagtacaccacaaatatatatatatatatatatatatatatatatataagtataaaagtttttatacaattttaactggctaaatgttaagagaaatgtttgttagaccatcttaacttatttacaaattgagagagaatgaaagagagaagaaataactgattgatttgatccattagtgtaataggaagaaaaatatgaaaacaaaataaaattattgattagttgtttaaaattttttattgtcaaaaaataatcatccaaaaattaatcttagtatcacttttaataaatttaccgtaaatcagtttgcaattttacttagtgggtttggttttttatggttgcatggattacacgtagtatgtatttggtcgcttaaattgtaggttcggattctgtcaccttttctattgttttgtgttgtctggtacagtggaaaccgttttgtgatgcccccgccatccctttaatgatctattttgtattttttatttatttaatcactcgttaaatcttttttaacattacttacttaatctttatagctacaataaattttatttttaattttaataatttaaaacattccattatagactatgaggacgaaaaaaatgtaattataagaacgaaaatatgatatttttaaactataaggaaagaacaaattgatgcaggacaaaatgagtaagaagcctatatttttgtttcaaaaaaagaaacctatatttcattagccctccgaatttgatggaatatcatttttgtactaaaacaatagtagtacacgcttatagcccaagatcatttctgaacctaaaagttaaaggctcaaactgttttcgtggattttattttcacctttttttttcctctttgtatttcatgtttttgtatttgttttttcaaaaatacatttttccaaaattaatatttggaacatatagtttaccaaaaagaaggggagtagtgggaaaaaaaagtgcgaatggaatcccactttacttgtcgtgcttgataattgatatattcgttttaatttttttgctttaattatgacagattctaacatgggtttgtttaattgattgtgaatgaaaatttttgtagttcgtggagtacaagaagacgatatacctagacggtgacatccaagtatttggaaacatagaccacttgtttgatctgcctgataattatttctatgcggtgatggattgtttctgcgagaagacttggagccacacccctcagttccagattgggtactgccaacagtgccctgataaggttcaatggccctctcactttggttccaaacctcctctatatttcaatgctggcatgtttgtttatgagcctaatctcgacacctaccgtgatcttctccaaactgtccaactcaccaagcccacttcttttgctgagcaggtatatatatgctcaattaatagcatgcttcacattaaaagaaaataaaataaaaaaaagttaaacatatgatttagtccatcagcatgtctagcattatgaaatttctcttatacggataaatgttactagtttggtccttagcactgttaaccctcctgtgtattcttaatttagttccataagtatagtgtattcttaatttagtctctctttgtaaggattggattaaaaaatttatacatacaggaaacaaattaaaaatatactacatgtataaggatatgcgttataacgtttgtatgtataatagggatgggtataatctagtttttgatatacagagactaaattgagaatttgttagaatttgtaatacatataacgaaaaaattaaatatttaaccaaaactaatttagcatatatgagtttcaaagtgtaattgtgaatttgttttcatgtgttggtaggactttctcaacatgtacttcaaggacaagtacaagccaataccgaacatgtacaaccttgtgctggccatgttgtggcgtcaccctgaaaatgttgaacttgataaagttcaagtggttcattactgtgctgctgtgagtgttcaccttctcactatagattcattgaataattaaatttttttgtttgatttttacttggtaataatgtttgttttttcatttatgttacacactataggggtctaagccttggaggttcactgggaaggaagagaacatggatagggaagatatcaagatgcttgtgaagaagtggtgggacatatatgaagatgagacactggactacaataacaactctgtcaacgtggaacgtttcacatcggcactattggatgctgggggctttcagtttgtgccagcaccttctgctgcctaa

SEQ ID NO: 43 - protein, 330 aa, Glycine max
MPPNITTVVANVTTEQLPKARGGSGRAFVTFLAGNGDYVKGVVGLAKGLRKAKSMYPLVVAVLPDVPEEHREILKSQGCIVREIEPVYPPENQTQFAMAYYVINYSKLRIWEFVEYKKTIYLDGDIQVFGNIDHLFDLPDNYFYAVMDCFCEKTWSHTPQFQIGYCQQCPDKVQWPSHFGSKPPLYFNAGMFVYEPNLDTYRDLLQTVQLTKPTSFAEQDFLNMYFKDKYKPIPNMYNLVLAMLWRHPENVELDKVQVVHYCAAGSKPWRFTGKEENMDREDIKMLVKKWWDIYEDETLDYNNNSVNVERFTSALLDAGGFQFVPAPSAA

SEQ ID NO: 44 - DNA, 2705 bp, synthetic construct
  source 1..2705: mol_type = other DNA
atgccacctaacatcaccaccgttgttgccaatgtcaccaccgagcaattacccaaggctcgtggaggaagtgggcgtgccttcgtgacctttcttgctgggaacggtgattacgtaaagggtgtcgtgggtttggccaaaggactgagaaaggccaaaagcatgtaccctttggtggttgctgtgttaccagatatcgtgagattctcaaatcccaaggttgcattgtcagggagattgaacctgtgtaccctcctgagaaccagacccagttcgccatggcctattatgtcatcaattactccaagctacgtatttgggaggtatacacatatcttaactcttttgttttttagtttagtacaccacaaatatatatatatatatatatatatatatatatataagtataaaagtttttatacaattttaactggctaaatgttaagagaaatgtttgttagaccatcttaacttatttacaaattgagagagaatgaaagagagaagaaataactgattgatttgatccattagtgtaataggaagaaaaatatgaaaacaaaataaaattattgattagttgtttaaaattttttattgtcaaaaaataatcatccaaaaattaatcttagtatcacttttaataaatttaccgtaaatcagtttgcaattttacttagtgggtttggttttttatggttgcatggattacacgtagtatgtatttggtcgcttaaattgtaggttcggattctgtcaccttttctattgttttgtgttgtctggtacagtggaaaccgttttgtgatgcccccgccatccctttaatgatctattttgtattttttatttatttaatcactcgttaaatcttttttaacattacttacttaatctttatagctacaataaattttatttttaattttaataatttaaaacattccattatagactatgaggacgaaaaaaatgtaattataagaacgaaaatatgatatttttaaactataaggaaagaacaaattgatgcaggacaaaatgagtaagaagcctatatttttgtttcaaaaaaagaaacctatatttcattagccctccgaatttgatggaatatcatttttgtactaaaacaatagtagtacacgcttatagcccaagatcatttctgaacctaaaagttaaaggctcaaactgttttcgtggattttattttcacctttttttttcctctttgtatttcatgtttttgtatttgttttttcaaaaatacatttttccaaaattaatatttggaacatatagtttaccaaaaagaaggggagtagtgggaaaaaaaagtgcgaatggaatcccactttacttgtcgtgcttgataattgatatattcgttttaatttttttgctttaattatgacagattctaacatgggtttgtttaattgattgtgaatgaaaatttttgtagttcgtggagtacaagaagacgatatacctagacggtgacatccaagtatttggaaacatagaccacttgtttgatctgcctgataattatttctatgcggtgatggattgtttctgcgagaagacttggagccacacccctcagttccagattgggtactgccaacagtgccctgataaggttcaatggccctctcactttggttccaaacctcctctatatttcaatgctggcatgtttgtttatgagcctaatctcgacacctaccgtgatcttctccaaactgtccaactcaccaagcccacttcttttgctgagcaggtatatatatgctcaattaatagcatgcttcacattaaaagaaaataaaataaaaaaaagttaaacatatgatttagtccatcagcatgtctagcattatgaaatttctcttatacggataaatgttactagtttggtccttagcactgttaaccctcctgtgtattcttaatttagttccataagtatagtgtattcttaatttagtctctctttgtaaggattggattaaaaaatttatacatacaggaaacaaattaaaaatatactacatgtataaggatatgcgttataacgtttgtatgtataatagggatgggtataatctagtttttgatatacagagactaaattgagaatttgttagaatttgtaatacatataacgaaaaaattaaatatttaaccaaaactaatttagcatatatgagtttcaaagtgtaattgtgaatttgttttcatgtgttggtaggactttctcaacatgtacttcaaggacaagtacaagccaataccgaacatgtacaaccttgtgctggccatgttgtggcgtcaccctgaaaatgttgaacttgataaagttcaagtggttcattactgtgctgctgtgagtgttcaccttctcactatagattcattgaataattaaatttttttgtttgatttttacttggtaataatgtttgttttttcatttatgttacacactataggggtctaagccttggaggttcactgggaaggaagagaacatggatagggaagatatcaagatgcttgtgaagaagtggtgggacatatatgaagatgagacactggactacaataacaactctgtcaacgtggaacgtttcacatcggcactattggatgctgggggctttcagtttgtgccagcaccttctgctgcctaa

SEQ ID NO: 45 - DNA, 2707 bp, synthetic construct
  source 1..2707: mol_type = other DNA
atgccacctaacatcaccaccgttgttgccaatgtcaccaccgagcaattacccaaggctcgtggaggaagtgggcgtgccttcgtgacctttcttgctgggaacggtgattacgtaaagggtgtcgtgggtttggccaaaggactgagaaaggccaaaagcatgtaccctttggtggttgctgtgttaccagatgtatcgtgagattctcaaatcccaaggttgcattgtcagggagattgaacctgtgtaccctcctgagaaccagacccagttcgccatggcctattatgtcatcaattactccaagctacgtatttgggaggtatacacatatcttaactcttttgttttttagtttagtacaccacaaatatatatatatatatatatatatatatatatataagtataaaagtttttatacaattttaactggctaaatgttaagagaaatgtttgttagaccatcttaacttatttacaaattgagagagaatgaaagagagaagaaataactgattgatttgatccattagtgtaataggaagaaaaatatgaaaacaaaataaaattattgattagttgtttaaaattttttattgtcaaaaaataatcatccaaaaattaatcttagtatcacttttaataaatttaccgtaaatcagtttgcaattttacttagtgggtttggttttttatggttgcatggattacacgtagtatgtatttggtcgcttaaattgtaggttcggattctgtcaccttttctattgttttgtgttgtctggtacagtggaaaccgttttgtgatgcccccgccatccctttaatgatctattttgtattttttatttatttaatcactcgttaaatcttttttaacattacttacttaatctttatagctacaataaattttatttttaattttaataatttaaaacattccattatagactatgaggacgaaaaaaatgtaattataagaacgaaaatatgatatttttaaactataaggaaagaacaaattgatgcaggacaaaatgagtaagaagcctatatttttgtttcaaaaaaagaaacctatatttcattagccctccgaatttgatggaatatcatttttgtactaaaacaatagtagtacacgcttatagcccaagatcatttctgaacctaaaagttaaaggctcaaactgttttcgtggattttattttcacctttttttttcctctttgtatttcatgtttttgtatttgttttttcaaaaatacatttttccaaaattaatatttggaacatatagtttaccaaaaagaaggggagtagtgggaaaaaaaagtgcgaatggaatcccactttacttgtcgtgcttgataattgatatattcgttttaatttttttgctttaattatgacagattctaacatgggtttgtttaattgattgtgaatgaaaatttttgtagttcgtggagtacaagaagacgatatacctagacggtgacatccaagtatttggaaacatagaccacttgtttgatctgcctgataattatttctatgcggtgatggattgtttctgcgagaagacttggagccacacccctcagttccagattgggtactgccaacagtgccctgataaggttcaatggccctctcactttggttccaaacctcctctatatttcaatgctggcatgtttgtttatgagcctaatctcgacacctaccgtgatcttctccaaactgtccaactcaccaagcccacttcttttgctgagcaggtatatatatgctcaattaatagcatgcttcacattaaaagaaaataaaataaaaaaaagttaaacatatgatttagtccatcagcatgtctagcattatgaaatttctcttatacggataaatgttactagtttggtccttagcactgttaaccctcctgtgtattcttaatttagttccataagtatagtgtattcttaatttagtctctctttgtaaggattggattaaaaaatttatacatacaggaaacaaattaaaaatatactacatgtataaggatatgcgttataacgtttgtatgtataatagggatgggtataatctagtttttgatatacagagactaaattgagaatttgttagaatttgtaatacatataacgaaaaaattaaatatttaaccaaaactaatttagcatatatgagtttcaaagtgtaattgtgaatttgttttcatgtgttggtaggactttctcaacatgtacttcaaggacaagtacaagccaataccgaacatgtacaaccttgtgctggccatgttgtggcgtcaccctgaaaatgttgaacttgataaagttcaagtggttcattactgtgctgctgtgagtgttcaccttctcactatagattcattgaataattaaatttttttgtttgatttttacttggtaataatgtttgttttttcatttatgttacacactataggggtctaagccttggaggttcactgggaaggaagagaacatggatagggaagatatcaagatgcttgtgaagaagtggtgggacatatatgaagatgagacactggactacaataacaactctgtcaacgtggaacgtttcacatcggcactattggatgctgggggctttcagtttgtgccagcaccttctgctgcctaa

SEQ ID NO: 46 - DNA, 2717 bp, synthetic construct
  source 1..2717: mol_type = other DNA
atgccacctaacatcaccaccgttgttgccaatgtcaccaccgagcaattacccaaggctcgtggaggaagtgggcgtgccttcgtgacctttcttgctgggaacggtgattacgtaaagggtgtcgtgggtttggccaaaggactgagaaaggccaaaagcatgtaccctttggtggttgctgtgttaccagatgttcctgagaacatcgtgagattctcaaatcccaaggttgcattgtcagggagattgaacctgtgtaccctcctgagaaccagacccagttcgccatggcctattatgtcatcaattactccaagctacgtatttgggaggtatacacatatcttaactcttttgttttttagtttagtacaccacaaatatatatatatatatatatatatatatatatataagtataaaagtttttatacaattttaactggctaaatgttaagagaaatgtttgttagaccatcttaacttatttacaaattgagagagaatgaaagagagaagaaataactgattgatttgatccattagtgtaataggaagaaaaatatgaaaacaaaataaaattattgattagttgtttaaaattttttattgtcaaaaaataatcatccaaaaattaatcttagtatcacttttaataaatttaccgtaaatcagtttgcaattttacttagtgggtttggttttttatggttgcatggattacacgtagtatgtatttggtcgcttaaattgtaggttcggattctgtcaccttttctattgttttgtgttgtctggtacagtggaaaccgttttgtgatgcccccgccatccctttaatgatctattttgtattttttatttatttaatcactcgttaaatcttttttaacattacttacttaatctttatagctacaataaattttatttttaattttaataatttaaaacattccattatagactatgaggacgaaaaaaatgtaattataagaacgaaaatatgatatttttaaactataaggaaagaacaaattgatgcaggacaaaatgagtaagaagcctatatttttgtttcaaaaaaagaaacctatatttcattagccctccgaatttgatggaatatcatttttgtactaaaacaatagtagtacacgcttatagcccaagatcatttctgaacctaaaagttaaaggctcaaactgttttcgtggattttattttcacctttttttttcctctttgtatttcatgtttttgtatttgttttttcaaaaatacatttttccaaaattaatatttggaacatatagtttaccaaaaagaaggggagtagtgggaaaaaaaagtgcgaatggaatcccactttacttgtcgtgcttgataattgatatattcgttttaatttttttgctttaattatgacagattctaacatgggtttgtttaattgattgtgaatgaaaatttttgtagttcgtggagtacaagaagacgatatacctagacggtgacatccaagtatttggaaacatagaccacttgtttgatctgcctgataattatttctatgcggtgatggattgtttctgcgagaagacttggagccacacccctcagttccagattgggtactgccaacagtgccctgataaggttcaatggccctctcactttggttccaaacctcctctatatttcaatgctggcatgtttgtttatgagcctaatctcgacacctaccgtgatcttctccaaactgtccaactcaccaagcccacttcttttgctgagcaggtatatatatgctcaattaatagcatgcttcacattaaaagaaaataaaataaaaaaaagttaaacatatgatttagtccatcagcatgtctagcattatgaaatttctcttatacggataaatgttactagtttggtccttagcactgttaaccctcctgtgtattcttaatttagttccataagtatagtgtattcttaatttagtctctctttgtaaggattggattaaaaaatttatacatacaggaaacaaattaaaaatatactacatgtataaggatatgcgttataacgtttgtatgtataatagggatgggtataatctagtttttgatatacagagactaaattgagaatttgttagaatttgtaatacatataacgaaaaaattaaatatttaaccaaaactaatttagcatatatgagtttcaaagtgtaattgtgaatttgttttcatgtgttggtaggactttctcaacatgtacttcaaggacaagtacaagccaataccgaacatgtacaaccttgtgctggccatgttgtggcgtcaccctgaaaatgttgaacttgataaagttcaagtggttcattactgtgctgctgtgagtgttcaccttctcactatagattcattgaataattaaatttttttgtttgatttttacttggtaataatgtttgttttttcatttatgttacacactataggggtctaagccttggaggttcactgggaaggaagagaacatggatagggaagatatcaagatgcttgtgaagaagtggtgggacatatatgaagatgagacactggactacaataacaactctgtcaacgtggaacgtttcacatcggcactattggatgctgggggctttcagtttgtgccagcaccttctgctgcctaa

SEQ ID NO: 47 - protein, 117 aa, synthetic construct
MPPNITTVVANVTTEQLPKARGGSGRAFVTFLAGNGDYVKGVVGLAKGLRKAKSMYPLVVAVLPDIVRFSNPKVALSGRLNLCTLLRTRPSSPWPIMSSITPSYVFGSSWSTRRRYT

SEQ ID NO: 48 - protein, 67 aa, synthetic construct
MPPNITTVVANVTTEQLPKARGGSGRAFVTFLAGNGDYVKGVVGLAKGLRKAKSMYPLVVAVLPDVS

SEQ ID NO: 49 - protein, 121 aa, synthetic construct
MPPNITTVVANVTTEQLPKARGGSGRAFVTFLAGNGDYVKGVVGLAKGLRKAKSMYPLVVAVLPDVPENIVRFSNPKVALSGRLNLCTLLRTRPSSPWPIMSSITPSYVFGSSWSTRRRYT

SEQ ID NO: 50 - DNA, 2898 bp, Glycine max
  source 1..2898: mol_type = genomic DNA
atggcacctaacatcaccaccgttgttgccaatgccaccactgagcaattacccaaagctcatggaggaagtagtgggcgtgcctttgtgacttttcttgctggaaacggtgattatgtaaagggtgttgtgggtttggccaaaggactgagaaaggccaaaagcatgtaccctttggtggttgctgtgttaccagatgttcctgaagaacatcgtgcgattctcaaatcccaaggttgcattgtcagggagattgaacctgtgtaccctcctaagaaccagacccagttcgccatggcctattatgtcatcaattactccaagctacgtatttgggaggtatatatatatatatatatatatatatatatatatatatatatatatatatatatatatatatatcttaaccttttctgtcaattggttttttagtttagtacacgtatcagtatagaagattttatacagttttaacggttgaaaattaatattagtatcacgattttaataaatttaccgtaaatcaagtttgtaattttacaaagtgggtttggttttttatggttgcgtgggttacacgtagtatgcattggtcgtttaatttggaggagtttgggagattctgtcaccttttctattgccttgtgttgtctggtacagtggaaaccgttttgtgatgccctctccaccctttcaataatcatttatattttttttatttaattagtcattaaatccttagagttacaaagctttttttttttctatagtttaaaacatttcaatattccctataattataagattttttttgtcctcgctttcaagtgttgaaaaaaattataattatagggaaaaaatatgttattttaaactatgaagacaaaaaaaaaaaatgattgcaggaacaaaatgaggaagaaaccgatattttatttgccctctgaatttgatggaataccatttttgtacttaaacaagtgtagtacacgtttatagctcaatataatttttgtacctaaaagttaaagtcccgaactgtttttaagataaaattagttaaaaatttacttgaaaattaaaaaaattagttagaagctgaaaacttaaaaattaatttattaaattaaaaatattcggtattaaaataactaaaaaatataaaatgatgaaaaaataatatcataatttattttaaaaagataataagaaaaatgaataaatatattaaagataaaaataaaaattagaaattaacgttttaaaaaatattagtttcagtaaagttttaaaaaaaatctacaagctcctaataaattattaaagcaagtttatttatgcaacaatcaaataaatttagcaaaaaaaattatctttatttgcacccttttattttctcttgcagtctttcatgttttgtattttttttagaaatactatttttcaaaaataaatttttggaatttaccaaaaagtagggtgtagtgaaaacaaaattatttttttatcaataaataatagtttattagtttcgttattgaaaacaaaatcatctgatccgagtttttttttttaattctgacatagtttagtttgatctatattgtgaatgaaattatttgcagttcgtggagtaccagaagatgatatacctagacggcgacatccaagtttttggaaacattgaccacttgtttgatcttcctaataattatttctatgcggtgatggattgtttctgcgagaagacttggagccacacccctcagttccagattgggtactgccaacagtgccctgataaggttcaatggccctctcactttggtaccaaacctcctctatatttcaatgctggcatgtttgtttatgagcctaatctcaacacctaccgtcatcttctccaaactgtccaagtcatcaagcccacgtcctttgctgagcaggtatatatttgctcaattaatagcatgcttcacatgaaaaaaaaaatataaagctacacatttaatttcattagtccagcaccatgtgtcgcattattaaattggtcttatgtgtaaatgttataagtttggtccttagcacggttaacctccttatgtattcttaatttagtttttattagtaagaattggattaaaattgcgtgttatacatgtaggaatcaaattaaaaatatactatacatgtatattgtataaggatatataaggggattatcctctgataacgtttgtatgtataaagtgatcgatttaatacactttttttttatatacagaaactaaattgcctataaaaagaaaagaaaaaagatatacaaagactaattaaattgagaatttgtaatacatatacataacaacaaaattatatatttaaccaaaaataaattagaatatgtgagtttcgaagtgtaattgtgaatttgttttcatgtacgtgtcgatataggactttctgaacatgtacttcaaggacaagtacaagccaataccgaacgtgtacaaccttgtgctggccatgttgtggcgtcaccctgagaatgttgaacttgatcaagttcaagtggttcattactgtgctgctgtaagtgttcatctcacaatagattcattaattaaacttttttgtttgatttttagttggtaatgttaatgattgatgtttcatttgtgttacacactataggggtctaagccttggaggttcactgggaaggaagagaacatggatagggaagatatcaagatgcttatgaagaagtggtgggacatatatgaagatgagacactggactacaataacaactctgtcaatgtggaacgtttcacatcagtactattggatgctgggggttttcagtttgtgccagcaccttctgctgcctaa

SEQ ID NO: 51 - protein, 331 aa, Glycine max
MAPNITTVVANATTEQLPKAHGGSSGRAFVTFLAGNGDYVKGVVGLAKGLRKAKSMYPLVVAVLPDVPEEHRAILKSQGCIVREIEPVYPPKNQTQFAMAYYVINYSKLRIWEFVEYQKMIYLDGDIQVFGNIDHLFDLPNNYFYAVMDCFCEKTWSHTPQFQIGYCQQCPDKVQWPSHFGTKPPLYFNAGMFVYEPNLNTYRHLLQTVQVIKPTSFAEQDFLNMYFKDKYKPIPNVYNLVLAMLWRHPENVELDQVQVVHYCAAGSKPWRFTGKEENMDREDIKMLMKKWWDIYEDETLDYNNNSVNVERFTSVLLDAGGFQFVPAPSAA

SEQ ID NO: 52 - DNA, 24 bp, synthetic construct
  source 1..24: mol_type = other DNA
agaatctcacgatgttcttcagga